European Patent Specification EP 3 380 522 B1, published November 8, 2023. Title: ANTIBODY MOLECULES TO APRIL AND USES THEREOF. Applicant: VISTERRA, INC. The sequence listing filed with the application follows.

SEQUENCE LISTING (346 sequences)

SEQ ID NO: 1 - protein, 8 aa, Artificial Sequence
  source: /note="Description of Artificial Sequence: Synthetic peptide"
GYSITSGY

SEQ ID NO: 2 - protein, 5 aa, Artificial Sequence
  source: /note="Description of Artificial Sequence: Synthetic peptide"
SYDGY

SEQ ID NO: 3 - protein, 11 aa, Artificial Sequence
  source: /note="Description of Artificial Sequence: Synthetic peptide"
YYDYEDWYFGV

SEQ ID NO: 4 - protein, 15 aa, Artificial Sequence
  source: /note="Description of Artificial Sequence: Synthetic peptide"
RASESVSIIGTNSIH

SEQ ID NO: 5 - protein, 7 aa, Artificial Sequence
  source: /note="Description of Artificial Sequence: Synthetic peptide"
HASNLET

SEQ ID NO: 6 - protein, 9 aa, Artificial Sequence
  source: /note="Description of Artificial Sequence: Synthetic peptide"
LQSRKIPYT

SEQ ID NO: 7 - protein, 6 aa, Artificial Sequence
  source: /note="Description of Artificial Sequence: Synthetic peptide"
SGYYWN

SEQ ID NO: 8 - protein, 16 aa, Artificial Sequence
  source: /note="Description of Artificial Sequence: Synthetic peptide"
YISYDGYNNYNPSLKN

SEQ ID NO: 9 - protein, 120 aa, Artificial Sequence
  source: /note="Description of Artificial Sequence: Synthetic polypeptide"
DVQLQESGPGLVKPSQSLSLTCSVTGYSITSGYYWNWIRQFPGNKLEWMGYISYDGYNNYNPSLKNRISITRDTSKNQFFLKLNSVTTEDTATYYCANYYDYEDWYFGVWGTGTTVTVSS

SEQ ID NO: 10 - protein, 111 aa, Artificial Sequence
  source: /note="Description of Artificial Sequence: Synthetic polypeptide"
DIVLTQSPASLAMSLGKRATISCRASESVSIIGTNSIHWYQQKPGQPPKLLIYHASNLETGVPARFSGSGSRTDFTLTIDPVEEDDVAIYYCLQSRKIPYTFGGGTKLEIK

SEQ ID NO: 11 - protein, 7 aa, Artificial Sequence
  source: /note="Description of Artificial Sequence: Synthetic peptide"
GYTFTDY

SEQ ID NO: 12 - protein, 6 aa, Artificial Sequence
  source: /note="Description of Artificial Sequence: Synthetic peptide"
YPLRGS

SEQ ID NO: 13 - protein, 11 aa, Artificial Sequence
  source: /note="Description of Artificial Sequence: Synthetic peptide"
HGAYYSNAFDY

SEQ ID NO: 14 - protein, 15 aa, Artificial Sequence
  source: /note="Description of Artificial Sequence: Synthetic peptide"
RASESVDNDGIRFMH

SEQ ID NO: 15 - protein, 7 aa, Artificial Sequence
  source: /note="Description of Artificial Sequence: Synthetic peptide"
RASNLES

SEQ ID NO: 16 - protein, 9 aa, Artificial Sequence
  source: /note="Description of Artificial Sequence: Synthetic peptide"
QQSNKDPYT

SEQ ID NO: 17 - protein, 5 aa, Artificial Sequence
  source: /note="Description of Artificial Sequence: Synthetic peptide"
DYTIH

SEQ ID NO: 18 - protein, 17 aa, Artificial Sequence
  source: /note="Description of Artificial Sequence: Synthetic peptide"
WIYPLRGSINYNEKFKD

SEQ ID NO: 19 - protein, 120 aa, Artificial Sequence
  source: /note="Description of Artificial Sequence: Synthetic polypeptide"
QVQLQQSGAELVKPGASVRLSCEASGYTFTDYTIHWVKQRSGQGLEWIGWIYPLRGSINYNEKFKDKATLTADKSSSTVYLELGRLTSKDSAVYFCARHGAYYSNAFDYWGQGTTLTVSS

SEQ ID NO: 20 - protein, 111 aa, Artificial Sequence
  source: /note="Description of Artificial Sequence: Synthetic polypeptide"
NIVMTQSPASLAVSLGQRATISCRASESVDNDGIRFMHWYQQKPGQPPKLLIYRASNLESGIPARFSGSGSRTDFTLTINPVETDDVATYYCQQSNKDPYTFGGGTKLELK

SEQ ID NO: 21 - protein, 7 aa, Artificial Sequence
  source: /note="Description of Artificial Sequence: Synthetic peptide"
GYTFTSY

SEQ ID NO: 22 - protein, 6 aa, Artificial Sequence
  source: /note="Description of Artificial Sequence: Synthetic peptide"
YIGNGY

SEQ ID NO: 23 - protein, 7 aa, Artificial Sequence
  source: /note="Description of Artificial Sequence: Synthetic peptide"
YYPWFTY

SEQ ID NO: 24 - protein, 11 aa, Artificial Sequence
  source: /note="Description of Artificial Sequence: Synthetic peptide"
RASENIYSYLA

SEQ ID NO: 25 - protein, 7 aa, Artificial Sequence
  source: /note="Description of Artificial Sequence: Synthetic peptide"
NAKTLAE

SEQ ID NO: 26 - protein, 9 aa, Artificial Sequence
  source: /note="Description of Artificial Sequence: Synthetic peptide"
QHHYDTPFT

SEQ ID NO: 27 - protein, 5 aa, Artificial Sequence
  source: /note="Description of Artificial Sequence: Synthetic peptide"
SYGIN

SEQ ID NO: 28 - protein, 17 aa, Artificial Sequence
  source: /note="Description of Artificial Sequence: Synthetic peptide"
YIYIGNGYAEYNERFKG

SEQ ID NO: 29 - protein, 116 aa, Artificial Sequence
  source: /note="Description of Artificial Sequence: Synthetic polypeptide"
EVQLQQSGAELVRPGSSVKMSCKTSGYTFTSYGINWVKQRPGQGLEWIGYIYIGNGYAEYNERFKGKATLTSDTSSSTAYMQLSSLTSEDSAIYFCALYYPWFTYWGQGTLVTVSA

SEQ ID NO: 30 - protein, 107 aa, Artificial Sequence
  source: /note="Description of Artificial Sequence: Synthetic polypeptide"
DIQMTQSPASLSASVGDSVTITCRASENIYSYLAWYQQKQGKSPQLLVYNAKTLAEGVPSRFSGSGSGTQFSLKINSLQPEDFGNYYCQHHYDTPFTFGGGTKLEIK

SEQ ID NO: 31 - skipped

SEQ ID NO: 32 - protein, 6 aa, Artificial Sequence
  source: /note="Description of Artificial Sequence: Synthetic peptide"
YPRDSS

SEQ ID NO: 33 - protein, 12 aa, Artificial Sequence
  source: /note="Description of Artificial Sequence: Synthetic peptide"
EGYDYDKRGFDY

SEQ ID NO: 34 - protein, 15 aa, Artificial Sequence
  source: /note="Description of Artificial Sequence: Synthetic peptide"
KASQSVSFAGTNLMH

SEQ ID NO: 35 - protein, 7 aa, Artificial Sequence
  source: /note="Description of Artificial Sequence: Synthetic peptide"
RASNLEP

SEQ ID NO: 36 - protein, 9 aa, Artificial Sequence
  source: /note="Description of Artificial Sequence: Synthetic peptide"
QQSREYPWT

SEQ ID NO: 37 - protein, 5 aa, Artificial Sequence
  source: /note="Description of Artificial Sequence: Synthetic peptide"
SYDVF

SEQ ID NO: 38 - protein, 17 aa, Artificial Sequence
  source: /note="Description of Artificial Sequence: Synthetic peptide"
WIYPRDSSTKYNEKFKG

SEQ ID NO: 39 - protein, 121 aa, Artificial Sequence
  source: /note="Description of Artificial Sequence: Synthetic polypeptide"
QVQLHQSGPELVKPGASVKLSCKTSGYTFTSYDVFWVKQRPGQGLEWIGWIYPRDSSTKYNEKFKGKATLTVDTSSSTAYMELHSLTSEDSAVYFCAKEGYDYDKRGFDYWGQGTTLTVSS

SEQ ID NO: 40 - protein, 111 aa, Artificial Sequence
  source: /note="Description of Artificial Sequence: Synthetic polypeptide"
DIVLTQSPASLAVSLGQRAIISCKASQSVSFAGTNLMHWYQQRPGQQPKLLIYRASNLEPGVPTRFSGSGSRTDFTLNIHPVEEDDAATYYCQQSREYPWTFGGGTKLEIK

SEQ ID NO: 41 - skipped

SEQ ID NO: 42 - protein, 6 aa, Artificial Sequence
  source: /note="Description of Artificial Sequence: Synthetic peptide"
DPETGG

SEQ ID NO: 43 - protein, 6 aa, Artificial Sequence
  source: /note="Description of Artificial Sequence: Synthetic peptide"
WNDGDY

SEQ ID NO: 44 - protein, 16 aa, Artificial Sequence
  source: /note="Description of Artificial Sequence: Synthetic peptide"
KSSQSLLYSNGKTYLN

SEQ ID NO: 45 - protein, 7 aa, Artificial Sequence
  source: /note="Description of Artificial Sequence: Synthetic peptide"
QVSKLDP

SEQ ID NO: 46 - protein, 9 aa, Artificial Sequence
  source: /note="Description of Artificial Sequence: Synthetic peptide"
LQGTYYPYT

SEQ ID NO: 47 - protein, 5 aa, Artificial Sequence
  source: /note="Description of Artificial Sequence: Synthetic peptide"
DYEMH

SEQ ID NO: 48 - protein, 17 aa, Artificial Sequence
  source: /note="Description of Artificial Sequence: Synthetic peptide"
AIDPETGGTAYNQRFKG

SEQ ID NO: 49 - protein, 115 aa, Artificial Sequence
  source: /note="Description of Artificial Sequence: Synthetic polypeptide"
QVQLQQSGAELVRPGASVTLSCKASGYTFTDYEMHWVKQTPVHGLEWIGAIDPETGGTAYNQRFKGKAILTTDKSSITAYMELRSLTSEDSAVYYCTRWNDGDYWGQGTTLTVSS

SEQ ID NO: 50 - protein, 112 aa, Artificial Sequence
  source: /note="Description of Artificial Sequence: Synthetic polypeptide"
DVVMTQTPLSLSVTIGQPASISCKSSQSLLYSNGKTYLNWFQQRPGQSPKRLMYQVSKLDPGIPDRFSGSGSETDFTLKISRVEAEDLGLYYCLQGTYYPYTFGGGTKLEIK

SEQ ID NO: 51 - protein, 7 aa, Artificial Sequence
  source: /note="Description of Artificial Sequence: Synthetic peptide"
GYSFTGY

SEQ ID NO: 52 - protein, 6 aa, Artificial Sequence
  source: /note="Description of Artificial Sequence: Synthetic peptide"
NPYNGD

SEQ ID NO: 53 - protein, 11 aa, Artificial Sequence
  source: /note="Description of Artificial Sequence: Synthetic peptide"
EGDGYYWYFDV

SEQ ID NO: 54 - protein, 15 aa, Artificial Sequence
  source: /note="Description of Artificial Sequence: Synthetic peptide"
RASESVDNYGISFMN

SEQ ID NO: 55 - protein, 7 aa, Artificial Sequence
  source: /note="Description of Artificial Sequence: Synthetic peptide"
AASNQGS

SEQ ID NO: 56 - protein, 9 aa, Artificial Sequence
  source: /note="Description of Artificial Sequence: Synthetic peptide"
QQSKEVPRT

SEQ ID NO: 57 - protein, 5 aa, Artificial Sequence
  source: /note="Description of Artificial Sequence: Synthetic peptide"
GYFMN

SEQ ID NO: 58 - protein, 17 aa, Artificial Sequence
  source: /note="Description of Artificial Sequence: Synthetic peptide"
RINPYNGDTFYNQKFKG

SEQ ID NO: 59 - protein, 120 aa, Artificial Sequence
  source: /note="Description of Artificial Sequence: Synthetic polypeptide"
EVQLQQSGPELVKPGASVKMSCKASGYSFTGYFMNWVKQSHGKSLEWIGRINPYNGDTFYNQKFKGKATLTVDKSSSTAHMELRSLTSEDSALYYCASEGDGYYWYFDVWGAGTTVTVSS

SEQ ID NO: 60 - protein, 111 aa, Artificial Sequence
  source: /note="Description of Artificial Sequence: Synthetic polypeptide"
DIVLTQSPASLAVSLGQRATISCRASESVDNYGISFMNWFQQKPGQPPKLLIYAASNQGSGVPARFSGSGSGTDFSLNIHPMEEDDTAMYFCQQSKEVPRTFGGGTKLEIK

SEQ ID NO: 61 - protein, 7 aa, Artificial Sequence
  source: /note="Description of Artificial Sequence: Synthetic peptide"
GYTFTDH

SEQ ID NO: 62 - protein, 6 aa, Artificial Sequence
  source: /note="Description of Artificial Sequence: Synthetic peptide"
DPDTGD

SEQ ID NO: 63 - protein, 6 aa, Artificial Sequence
  source: /note="Description of Artificial Sequence: Synthetic peptide"
WTGGDY

SEQ ID NO: 64 - protein, 5 aa, Artificial Sequence
  source: /note="Description of Artificial Sequence: Synthetic peptide"
DHEMH

SEQ ID NO: 65 - protein, 17 aa, Artificial Sequence
  source: /note="Description of Artificial Sequence: Synthetic peptide"
VIDPDTGDTTYNQKFKG

SEQ ID NO: 66 - protein, 115 aa, Artificial Sequence
  source: /note="Description of Artificial Sequence: Synthetic polypeptide"
QVQLQQSGAELVRPGASVKLSCKASGYTFTDHEMHWVRQTPVHGLEWIGVIDPDTGDTTYNQKFKGKATLTADKSSSTAYMDLRSLTSEDSAVFYCTRWTGGDYWGHGTTLTVSS

SEQ ID NO: 67 - protein, 16 aa, Artificial Sequence
  source: /note="Description of Artificial Sequence: Synthetic peptide"
KSSQSLLYSDGKTYLN

SEQ ID NO: 68-69 - skipped (2 entries)

SEQ ID NO: 70 - protein, 112 aa, Artificial Sequence
  source: /note="Description of Artificial Sequence: Synthetic polypeptide"
DAVMTQTPLSLSVTIGQPASISCKSSQSLLYSDGKTYLNWFQQRPGQSPKRLMYQVSKLDPGIPDRFSGSGSETDFTLKISRVEAEDLGVYYCLQGTYYPYTFGSGTKLEIK

SEQ ID NO: 71 - DNA, 360 bp, Artificial Sequence
  source: /note="Description of Artificial Sequence: Synthetic polynucleotide"
gatgtacagcttcaggagtcaggacctggcctcgtgaaaccttctcagtctctgtctctcacctgctctgtcactggctactccatcaccagtggttattactggaactggatccggcagtttccaggaaacaaactggaatggatgggctacataagctacgatggttacaataactacaacccatctctcaaaaatcgaatctccatcactcgtgacacatctaagaaccagtttttcctgaagttgaattctgtgactactgaggacacagccacatattactgtgcaaactactatgattacgaagactggtacttcggtgtctggggcacagggaccacggtcaccgtctcctca

SEQ ID NO: 72 - DNA, 333 bp, Artificial Sequence
  source: /note="Description of Artificial Sequence: Synthetic polynucleotide"
gacattgtgctgacccaatctccagcttctttggctatgtctctagggaagagggccaccatctcctgcagagccagcgaaagtgtcagtattattggtactaattcaatacactggtaccaacagaaaccaggacagccacccaaactcctcatctatcatgcatccaacctagaaactggagtccctgccaggttcagtggcagtgggtctagaacagacttcaccctcaccattgatcctgtggaggaagatgatgttgcaatctattactgtctgcaaagtaggaagattccgtacacgttcggaggggggaccaagctggaaataaaa

SEQ ID NO: 73 - DNA, 360 bp, Artificial Sequence
  source: /note="Description of Artificial Sequence: Synthetic polynucleotide"
caggtccagctgcagcagtctggagctgagctggtgaaacccggggcatcagtgaggctgtcctgcgaggcttctggctacaccttcacggactatactatacactgggtaaagcagaggtctggacagggtcttgagtggattggatggatttaccctctaagaggtagtataaactacaatgagaaattcaaggacaaggccacattgactgcggacaaatcctccagcacagtctatttggagcttggtagattgacatctaaggactctgcggtctatttctgtgcaagacacggagcctactatagtaacgcctttgactactggggccaaggcaccactctcacagtctcctca

SEQ ID NO: 74 - DNA, 333 bp, Artificial Sequence
  source: /note="Description of Artificial Sequence: Synthetic polynucleotide"
aacattgtaatgacccaatctccagcttcattggctgtgtctctaggtcagagggccaccatctcctgcagagccagcgagagtgttgataatgatggcattagatttatgcactggtaccagcagaaaccaggacagccacccaaactcctcatctatcgtgcatccaacctagaatctgggatccctgccaggttcagtggcagtgggtctaggacagacttcaccctcactattaatcctgtggagactgatgatgttgcaacctattactgtcagcaaagtaataaggatccgtacacgttcggaggggggaccaagctggagctgaaa

SEQ ID NO: 75 - DNA, 348 bp, Artificial Sequence
  source: /note="Description of Artificial Sequence: Synthetic polynucleotide"
gaggtccagcttcagcagtctggagctgagctggtgaggcctgggtcctcagtgaagatgtcctgcaagacttctggatatactttcacaagctacggtataaactgggtgaagcagaggcctggacagggcctggaatggattggatatatttatattggaaatggttatgctgagtacaatgagaggttcaagggcaaggccacactgacttcagacacatcctccagcacagcctacatgcagctcagcagcctgacatctgaggactctgcaatctatttctgtgcactatactatccctggtttacttactggggccaggggactctggtcactgtctctgca

SEQ ID NO: 76 - DNA, 321 bp, Artificial Sequence
  source: /note="Description of Artificial Sequence: Synthetic polynucleotide"
gacatccagatgactcagtctccagcctccctttctgcatctgtgggagattctgtcaccatcacatgtcgagcaagtgagaatatttacagttatttagcatggtatcagcagaaacagggaaaatctcctcagctcctggtctataatgcaaaaaccttagctgaaggtgtgccatcaaggttcagtggcagtggatcaggcacacagttttctctgaagatcaacagcctgcagcctgaagattttgggaattattactgtcaacatcattatgatactccgttcacgttcggaggggggaccaagctggaaataaaa

SEQ ID NO: 77 - DNA, 363 bp, Artificial Sequence
  source: /note="Description of Artificial Sequence: Synthetic polynucleotide"
caggttcagctgcaccagtctggacctgagctggtgaagcctggggcttcagtgaagttgtcctgcaagacttctggctacaccttcacaagctacgatgtcttctgggtgaagcagaggcctggacagggacttgagtggattggatggatttatcctagagatagtagtactaaatacaatgagaagttcaagggcaaggccacattgactgtagacacatcctccagcacagcatacatggagctccacagcctgacatctgaggactctgcggtctatttctgtgcaaaagaggggtatgattatgacaagaggggctttgactactggggccaaggcaccactctcacagtctcctca

SEQ ID NO: 78 - DNA, 333 bp, Artificial Sequence
  source: /note="Description of Artificial Sequence: Synthetic polynucleotide"
gacattgtgctgacccaatctccagcttctttggctgtgtctctagggcagagggccatcatctcctgcaaggccagccaaagtgtcagttttgctggtactaatttaatgcactggtaccaacagagaccagggcagcaacccaaactcctcatctatcgtgcatccaacctagaacctggggttcctaccaggtttagtggcagtgggtctaggacagacttcaccctcaatatccatcctgtggaggaagatgatgctgcaacctattactgtcagcaaagtagggaatatccgtggacgttcggtggaggcaccaagctggaaatcaaa

SEQ ID NO: 79 - DNA, 345 bp, Artificial Sequence
  source: /note="Description of Artificial Sequence: Synthetic polynucleotide"
caggttcaactgcagcagtctggggctgagctggtgaggcctggggcttcagtgacgctgtcctgcaaggcttcgggctacacttttactgactatgaaatgcactgggtgaagcagacacctgtgcatggcctggaatggattggagctattgatcctgaaactggtggtactgcctacaatcagaggttcaagggcaaggccatactgactacagacaaatcctccatcacagcctacatggagctccgcagcctgacatctgaggactctgccgtctattactgtacaagatggaatgatggcgactactggggccaaggcaccactctcacagtctcctca

SEQ ID NO: 80 - DNA, 336 bp, Artificial Sequence
  source: /note="Description of Artificial Sequence: Synthetic polynucleotide"
gatgttgtgatgacccagactccactgtctttgtcggttaccattggacaaccagcctccatttcttgcaagtcaagtcagagcctcttatacagtaatggaaagacatatttgaattggtttcaacagaggcctggccagtctccaaagcgcctaatgtatcaggtgtccaaactggaccctggcatccctgacaggttcagtggcagtggatcagaaacagattttacacttaaaatcagcagagtggaggctgaagatttgggactttattactgcttgcaaggtacatattatccgtacacgttcggaggggggaccaagctggaaataaaa

SEQ ID NO: 81 - DNA, 360 bp, Artificial Sequence
  source: /note="Description of Artificial Sequence: Synthetic polynucleotide"
gaggtccagctgcagcagtctggacctgagctggtgaagcctggggcttcagtgaagatgtcctgcaaggcttctggttactcctttactggctactttatgaactgggtgaagcagagccatggaaagagccttgagtggattggacgtattaatccttacaatggtgatactttctacaaccagaagttcaagggcaaggccacattgactgtagacaaatcctctagcacagcccacatggagctccggagcctgacatctgaggactctgcactctattattgtgcaagcgaaggtgatggttactactggtacttcgatgtctggggcgcagggaccacggtcaccgtctcctca

SEQ ID NO: 82 - DNA, 333 bp, Artificial Sequence
  source: /note="Description of Artificial Sequence: Synthetic polynucleotide"
gacattgtgctgacccaatctccagcttctttggctgtgtctctagggcagagggccaccatctcctgcagagccagcgaaagtgttgataattatggcattagttttatgaactggttccaacagaaaccaggacagccacccaaactcctcatctatgctgcatccaaccaaggatccggggtccctgccaggtttagtggcagtgggtctgggacagacttcagcctcaacatccatcctatggaggaggatgatactgcaatgtatttctgtcagcaaagtaaggaggttcctcggacgttcggtggaggcaccaagctggaaatcaaa

SEQ ID NO: 83 - DNA, 345 bp, Artificial Sequence
  source: /note="Description of Artificial Sequence: Synthetic polynucleotide"
caggttcaactgcagcagtctggggctgagctggtgaggcctggggcttcagtgaagctgtcctgcaaggcttcgggctacacatttactgaccatgaaatgcactgggtgagacagacacctgtgcatggcctggaatggattggagttattgatcctgacactggtgatactacctacaatcagaaattcaagggcaaggccacactgactgcagacaaatcctccagcacagcctacatggacctccgcagcctgacatctgaggactctgccgtcttttactgtacacggtggactgggggggactactggggccatggcaccactctcacagtctcctca

SEQ ID NO: 84 - DNA, 336 bp, Artificial Sequence
  source: /note="Description of Artificial Sequence: Synthetic polynucleotide"
gatgctgtgatgacccagactccactgtctttgtcggttaccattggacaaccagcctctatctcttgcaagtcgagtcagagcctcttatatagtgatggaaagacatatttgaattggttccaacagaggccaggccagtctccaaagcgcctaatgtatcaggtgtccaaactggaccctggcatccctgacaggttcagtggcagtggatcagagacagattttacacttaaaatcagcagagtggaggctgaggatttgggagtttattactgcttgcaaggtacatattatccgtatacgttcggatcggggaccaagctggaaataaaa

SEQ ID NO: 85 - protein, 250 aa, Homo sapiens [sequence omitted]

SEQ ID NO: 86 - protein, 234 aa, Homo sapiens
MPASSPFLLAPKGPPGNMGGPVREPALSVALWLSWGAALGAVACAMALLTQQTELQSLRREVSRLQGTGGPSQNGEGYPWQSLPEQSSDALEAWENGERSRKRRAVLTQKQKNDSDVTEVMWQPALRRGRGLQAQGYGVRIQDAGVYLLYSQVLFQDVTFTMGQVVSREGQGRQETLFRCIRSMPSHPDRAYNSCYSAGVFHLHQGDILSVIIPRARAKLNLSPHGTFLGFVKL

SEQ ID NO: 87 - protein, 247 aa, Homo sapiens
MPASSPFLLAPKGPPGNMGGPVREPALSVALWLSWGAALGAVACAMALLTQQTELQSLRREVSRLQGTGGPSQNGEGYPWQSLPEQSSDALEAWENGERSRKRRAVLTQKQKKQHSVLHLVPINATSKDDSDVTEVMWQPALRRGRGLQAQGYGVRIQDAGVYLLYSQVLFQDVTFTMGQVVSREGQGRQETLFRCIRSMPSHPDRAYNSCYSAGVFHLHQGDILSVIIPRARAKLNLSPHGTFLGL

SEQ ID NO: 88 - protein, 222 aa, Homo sapiens
MPASSPFLLAPKGPPGNMGGPVREPALSVALWLSWGAALGAVACAMALLTQQTELQSLRREVSRLQGTGGPSQNGEGYPWQSLPEQHSVLHLVPINATSKDDSDVTEVMWQPALRRGRGLQAQGYGVRIQDAGVYLLYSQVLFQDVTFTMGQVVSREGQGRQETLFRCIRSMPSHPDRAYNSCYSAGVFHLHQGDILSVIIPRARAKLNLSPHGTFLGFVKL

SEQ ID NO: 89 - protein, 330 aa, Homo sapiens
MAARRSQRRRGRRGEPGTALLVPLALGLGLALACLGLLLAVVSLGSRASLSAQEPAQEELVAEEDQDPSELNPQTEESQDPAPFLNRLVRPRRSAPKGRKTRARRAIAAHYEVHPRPGQDGAQAGVDGTVSGWEEARINSSSPLRYNRQIGEFIVTRAGLYYLYCQSSDALEAWENGERSRKRRAVLTQKQKKQHSVLHLVPINATSKDDSDVTEVMWQPALRRGRGLQAQGYGVRIQDAGVYLLYSQVLFQDVTFTMGQVVSREGQGRQETLFRCIRSMPSHPDRAYNSCYSAGVFHLHQGDILSVIIPRARAKLNLSPHGTFLGFVKL

SEQ ID NO: 90 - protein, 205 aa, Homo sapiens
MGGPVREPALSVALWLSWGAALGAVACAMALLTQQTELQSLRREVSRLQGTGGPSQNGEGYPWQSLPEQHSVLHLVPINATSKDDSDVTEVMWQPALRRGRGLQAQGYGVRIQDAGVYLLYSQVLFQDVTFTMGQVVSREGQGRQETLFRCIRSMPSHPDRAYNSCYSAGVFHLHQGDILSVIIPRARAKLNLSPHGTFLGFVKL

SEQ ID NO: 91 - protein, 241 aa, Mus musculus
MPASSPGHMGGSVREPALSVALWLSWGAVLGAVTCAVALLIQQTELQSLRREVSRLQRSGGPSQKQGERPWQSLWEQSPDVLEAWKDGAKSRRRRAVLTQKHKKKHSVLHLVPVNITSKADSDVTEVMWQPVLRRGRGLEAQGDIVRVWDTGIYLLYSQVLFHDVTFTMGQVVSREGQGRRETLFRCIRSMPSDPDRAYNSCYSAGVFHLHQGDIITVKIPRANAKLSLSPHGTFLGFVKL

SEQ ID NO: 92 - protein, 240 aa, Mus musculus
MPASSPGHMGGSVREPALSVALWLSWGAVLGAVTCAVALLIQQTELQSLRREVSRLQRSGGPSQKQGERPWQSLWEQSPDVLEAWKDGAKSRRRRAVLTQKHKKKHSVLHLVPVNITSKDSDVTEVMWQPVLRRGRGLEAQGDIVRVWDTGIYLLYSQVLFHDVTFTMGQVVSREGQGRRETLFRCIRSMPSDPDRAYNSCYSAGVFHLHQGDIITVKIPRANAKLSLSPHGTFLGFVKL

SEQ ID NO: 93 - protein, 7 aa, Artificial Sequence
  source: /note="Description of Artificial Sequence: Synthetic peptide"
GFSLTIY

SEQ ID NO: 94 - protein, 5 aa, Artificial Sequence
  source: /note="Description of Artificial Sequence: Synthetic peptide"
WSDGS

SEQ ID NO: 95 - protein, 10 aa, Artificial Sequence
  source: /note="Description of Artificial Sequence: Synthetic peptide"
NWVDQAWFAY

SEQ ID NO: 96 - protein, 11 aa, Artificial Sequence
  source: /note="Description of Artificial Sequence: Synthetic peptide"
RASKNIYSYLA

SEQ ID NO: 97 - protein, 7 aa, Artificial Sequence
  source: /note="Description of Artificial Sequence: Synthetic peptide"
NAKTLPE

SEQ ID NO: 98 - protein, 9 aa, Artificial Sequence
  source: /note="Description of Artificial Sequence: Synthetic peptide"
QHHYGTPLT

SEQ ID NO: 99 - protein, 5 aa, Artificial Sequence
  source: /note="Description of Artificial Sequence: Synthetic peptide"
IYDVH

SEQ ID NO: 100 - protein, 16 aa, Artificial Sequence
  source: /note="Description of Artificial Sequence: Synthetic peptide"
VIWSDGSTDYNAAFIS

SEQ ID NO: 101 - protein, 118 aa, Artificial Sequence
  source: /note="Description of Artificial Sequence: Synthetic polypeptide"
QVQLKESGPGLVAPSQSLSITCTVSGFSLTIYDVHWVRQSPGKGLEWLGVIWSDGSTDYNAAFISRLSISKDNSKSQVFFKMNSLQADDTAIYYCARNWVDQAWFAYWGQGTLVTVSA

SEQ ID NO: 102 - protein, 107 aa, Artificial Sequence
  source: /note="Description of Artificial Sequence: Synthetic polypeptide"
DIQMTQSPASLSASVGETITITCRASKNIYSYLAWYQQKQGKSPQLLVYNAKTLPEGVPSRFSGSGSGTQFSLKINSLQPEDFGSYYCQHHYGTPLTFGAGTKLELK

SEQ ID NO: 103 - protein, 7 aa, Artificial Sequence
  source: /note="Description of Artificial Sequence: Synthetic peptide"
GYIFTDY

SEQ ID NO: 104 - protein, 6 aa, Artificial Sequence
  source: /note="Description of Artificial Sequence: Synthetic peptide"
YPGSGN

SEQ ID NO: 105 - protein, 12 aa, Artificial Sequence
  source: /note="Description of Artificial Sequence: Synthetic peptide"
ESNYVGYYAMDY

SEQ ID NO: 106 - protein, 16 aa, Artificial Sequence
  source: /note="Description of Artificial Sequence: Synthetic peptide"
RSSQSVVNSNGNTYLE

SEQ ID NO: 107 - protein, 7 aa, Artificial Sequence
  source: /note="Description of Artificial Sequence: Synthetic peptide"
KVSNRFS

SEQ ID NO: 108 - protein, 9 aa, Artificial Sequence
  source: /note="Description of Artificial Sequence: Synthetic peptide"
FQGSHVPWT

SEQ ID NO: 109 - protein, 5 aa, Artificial Sequence
  source: /note="Description of Artificial Sequence: Synthetic peptide"
DYTIN

SEQ ID NO: 110 - protein, 17 aa, Artificial Sequence
  source: /note="Description of Artificial Sequence: Synthetic peptide"
WIYPGSGNRKYNDKFKG

SEQ ID NO: 111 - protein, 121 aa, Artificial Sequence
  source: /note="Description of Artificial Sequence: Synthetic polypeptide"
QVQLQQSGPELVKPGASVKLSCKAAGYIFTDYTINWVKQSPGQGLEWIGWIYPGSGNRKYNDKFKGKATMTADKSSSTAYMQLSSLTSEDSAVYFCARESNYVGYYAMDYWGQGTSVTVSS

SEQ ID NO: 112 - protein, 112 aa, Artificial Sequence
  source: /note="Description of Artificial Sequence: Synthetic polypeptide"
DVLMTQTPLSLPVSLGDQASISCRSSQSVVNSNGNTYLEWYLQKPGQSPNLLIYKVSNRFSGVPDRFSGSGSGTDFTLKISRVEAEDLGVYYCFQGSHVPWTFGGGTKLEIK

SEQ ID NO: 113 - protein, 7 aa, Artificial Sequence
  source: /note="Description of Artificial Sequence: Synthetic peptide"
GYTFTNY

SEQ ID NO: 114 - protein, 9 aa, Artificial Sequence
  source: /note="Description of Artificial Sequence: Synthetic peptide"
YPGGIGGGY

SEQ ID NO: 115 - protein, 9 aa, Artificial Sequence
  source: /note="Description of Artificial Sequence: Synthetic peptide"
SETGRAMDY

SEQ ID NO: 116 - protein, 11 aa, Artificial Sequence
  source: /note="Description of Artificial Sequence: Synthetic peptide"
KASQDINKYIA

SEQ ID NO: 117 - protein, 7 aa, Artificial Sequence
  source: /note="Description of Artificial Sequence: Synthetic peptide"
YTSTLKP

SEQ ID NO: 118 - protein, 8 aa, Artificial Sequence
  source: /note="Description of Artificial Sequence: Synthetic peptide"
LQYDNLNT

SEQ ID NO: 119 - protein, 5 aa, Artificial Sequence
  source: /note="Description of Artificial Sequence: Synthetic peptide"
NYWIG

SEQ ID NO: 120 - protein, 20 aa, Artificial Sequence
  source: /note="Description of Artificial Sequence: Synthetic peptide"
DIYPGGIGGGYTKYNEKFKG

SEQ ID NO: 121 - protein, 121 aa, Artificial Sequence
  source: /note="Description of Artificial Sequence: Synthetic polypeptide"
QVQLQQSGAELVRPGTSVKMSCKAAGYTFTNYWIGWVKQRPGHGLEWIGDIYPGGIGGGYTKYNEKFKGKATLTADTSSSTAYMQLGSLTSEDSAIYFCSRSETGRAMDYWGQGTSVTVSS

SEQ ID NO: 122 - protein, 106 aa, Artificial Sequence
  source: /note="Description of Artificial Sequence: Synthetic polypeptide"
DIQMTQSPSSLSASLGGKVTITCKASQDINKYIAWYQHKPGKGPRLLIHYTSTLKPGIPSRFSGSGSGRDYSFSISDLEPEDIATYYCLQYDNLNTFGGGTKLEIK

SEQ ID NO: 123 - protein, 7 aa, Artificial Sequence
  source: /note="Description of Artificial Sequence: Synthetic peptide"
GYSFTDY

SEQ ID NO: 124 - protein, 6 aa, Artificial Sequence
  source: /note="Description of Artificial Sequence: Synthetic peptide"
DPSNGG

SEQ ID NO: 125 - protein, 11 aa, Artificial Sequence
  source: /note="Description of Artificial Sequence: Synthetic peptide"
RDNYGSGTMDY

SEQ ID NO: 126 - protein, 11 aa, Artificial Sequence
  source: /note="Description of Artificial Sequence: Synthetic peptide"
KASQNVGTDVS

SEQ ID NO: 127 - protein, 7 aa, Artificial Sequence
  source: /note="Description of Artificial Sequence: Synthetic peptide"
WASNRFT

SEQ ID NO: 128 - protein, 9 aa, Artificial Sequence
  source: /note="Description of Artificial Sequence: Synthetic peptide"
EQYSIYPLT

SEQ ID NO: 129 - protein, 5 aa, Artificial Sequence
  source: /note="Description of Artificial Sequence: Synthetic peptide"
DYNIY

SEQ ID NO: 130 - protein, 17 aa, Artificial Sequence
  source: /note="Description of Artificial Sequence: Synthetic peptide"
YIDPSNGGPGYNQKFRG

SEQ ID NO: 131 - protein, 120 aa, Artificial Sequence
  source: /note="Description of Artificial Sequence: Synthetic polypeptide"
EIQLQQSGPELVKPGASVKVSCKASGYSFTDYNIYWVKQSHGKSLEWIGYIDPSNGGPGYNQKFRGKATLTVDKSSSTAFLHLNSLTSEDSAVYYCARRDNYGSGTMDYWGQGTSVTVSS

SEQ ID NO: 132 - protein, 107 aa, Artificial Sequence
  source: /note="Description of Artificial Sequence: Synthetic polypeptide"
DIVMTQSQKFMSTSVGDRVSITCKASQNVGTDVSWYQQKPGKSPKPLIYWASNRFTGVPDRFIGSGSGTDFTLTISNVQSEDLADYFCEQYSIYPLTFGAGTKLELK

SEQ ID NO: 133 - protein, 7 aa, Artificial Sequence
  source: /note="Description of Artificial Sequence: Synthetic peptide"
GYSFTDD

SEQ ID NO: 134 - protein, 6 aa, Artificial Sequence
  source: /note="Description of Artificial Sequence: Synthetic peptide"
DPLNGG

SEQ ID NO: 135 - protein, 11 aa, Artificial Sequence
  source: /note="Description of Artificial Sequence: Synthetic peptide"
RDNYATGTMDY

SEQ ID NO: 136 - protein, 11 aa, Artificial Sequence
  source: /note="Description of Artificial Sequence: Synthetic peptide"
KASKNVGTDVS

SEQ ID NO: 137 - protein, 9 aa, Artificial Sequence
  source: /note="Description of Artificial Sequence: Synthetic peptide"
EQYSSYPLT

SEQ ID NO: 138 - protein, 5 aa, Artificial Sequence
  source: /note="Description of Artificial Sequence: Synthetic peptide"
DDNMY

SEQ ID NO: 139 - protein, 17 aa, Artificial Sequence
  source: /note="Description of Artificial Sequence: Synthetic peptide"
YIDPLNGGTGYNQKFKG

SEQ ID NO: 140 - protein, 120 aa, Artificial Sequence
  source: /note="Description of Artificial Sequence: Synthetic polypeptide"
EIQLQQSGPELVKPGASVKVSCKASGYSFTDDNMYWVKQSHGKSLEWIGYIDPLNGGTGYNQKFKGKATLTVDKSSSTAFLHLNSLTSEDSAVYYCARRDNYATGTMDYWGQGTSVTVSS

SEQ ID NO: 141 - protein, 107 aa, Artificial Sequence
  source: /note="Description of Artificial Sequence: Synthetic polypeptide"
DIVMTQSQKFMSTSVGDRVSITCKASKNVGTDVSWYQQKPGKSPKPLIYWASNRFTGVPDRFTGSGSGTDFTLTINNVQSEDLADYFCEQYSSYPLTFGAGTKLELK

SEQ ID NO: 142 - protein, 6 aa, Artificial Sequence
  source: /note="Description of Artificial Sequence: Synthetic peptide"
YPINGY

SEQ ID NO: 143 - protein, 11 aa, Artificial Sequence
  source: /note="Description of Artificial Sequence: Synthetic peptide"
DSNYVGWYFDV

SEQ ID NO: 144 - protein, 16 aa, Artificial Sequence
  source: /note="Description of Artificial Sequence: Synthetic peptide"
RSSQSLVHSNGNTYLH

SEQ ID NO: 145 - protein, 9 aa, Artificial Sequence
  source: /note="Description of Artificial Sequence: Synthetic peptide"
SQSTHVPRT

SEQ ID NO: 146 - protein, 15 aa, Artificial Sequence
  source: /note="Description of Artificial Sequence: Synthetic peptide"
RASKSVSTSGYSYMH

SEQ ID NO: 147 - protein, 7 aa, Artificial Sequence
  source: /note="Description of Artificial Sequence: Synthetic peptide"
FTSDLEP

SEQ ID NO: 148 - protein, 9 aa, Artificial Sequence
  source: /note="Description of Artificial Sequence: Synthetic peptide"
QHSRELPYP

SEQ ID NO: 149 - protein, 5 aa, Artificial Sequence
  source: /note="Description of Artificial Sequence: Synthetic peptide"
DYNMD

SEQ ID NO: 150 - protein, 17 aa, Artificial Sequence
  source: /note="Description of Artificial Sequence: Synthetic peptide"
NIYPINGYTGYNQRFKN

SEQ ID NO: 151 - protein, 120 aa, Artificial Sequence
  source: /note="Description of Artificial Sequence: Synthetic polypeptide"
EVQLQQSGPELVKPGASVKISCKASGYTFTDYNMDWVKQSHGKSLEWIGNIYPINGYTGYNQRFKNKATLTVDKSSSTAYMELHSLTSEDSAVYYCARDSNYVGWYFDVWGAGTTVTVSS

SEQ ID NO: 152 - protein, 112 aa, Artificial Sequence
  source: /note="Description of Artificial Sequence: Synthetic polypeptide"
DVVMTQTPLSLPVSLGDQASISCRSSQSLVHSNGNTYLHWYLQKPGQSPKLLIYKVSNRFSGVPDRFSGSGSGTDFTFKISRVEAEDLGVYFCSQSTHVPRTFGGGTKLEIK

SEQ ID NO: 153 - protein, 111 aa, Artificial Sequence
  source: /note="Description of Artificial Sequence: Synthetic polypeptide"
DIVLTQSPASLTVSLGQRATFSCRASKSVSTSGYSYMHWYQQKPGQPPKLLIYFTSDLEPGVPARFTGSGSGTDFTLNIHPVEEEDAATYYCQHSRELPYPFGGGTKLEIK

SEQ ID NO: 154 - protein, 7 aa, Artificial Sequence
  source: /note="Description of Artificial Sequence: Synthetic peptide"
GYTFADY

SEQ ID NO: 155 - protein, 6 aa, Artificial Sequence
  source: /note="Description of Artificial Sequence: Synthetic peptide"
FPGSGS

SEQ ID NO: 156 - protein, 9 aa, Artificial Sequence
  source: /note="Description of Artificial Sequence: Synthetic peptide"
GDSGRAMDY

SEQ ID NO: 157 - protein, 7 aa, Artificial Sequence
  source: /note="Description of Artificial Sequence: Synthetic peptide"
YTSTLQS

SEQ ID NO: 158 - protein, 8 aa, Artificial Sequence
  source: /note="Description of Artificial Sequence: Synthetic peptide"
LQYDNLLT

SEQ ID NO: 159 - protein, 5 aa, Artificial Sequence
  source: /note="Description of Artificial Sequence: Synthetic peptide"
DYYIN

SEQ ID NO: 160 - protein, 17 aa, Artificial Sequence
  source: /note="Description of Artificial Sequence: Synthetic peptide"
WIFPGSGSTYYNEKFKG

SEQ ID NO: 161 - protein, 118 aa, Artificial Sequence
  source: /note="Description of Artificial Sequence: Synthetic polypeptide"
QVQLQQSGPELVKPGASVKISCKASGYTFADYYINWVKQRPGQGLEWIGWIFPGSGSTYYNEKFKGKATLTVDKSSSTAYMLLSSLTSEDSAVYFCARGDSGRAMDYWGQGTSVTVSS

SEQ ID NO: 162 - protein, 106 aa, Artificial Sequence
  source: /note="Description of Artificial Sequence: Synthetic polypeptide"
DIQMTQSPSSLSASLGGKVTITCKASQDINKYIAWYQHKPGKGPRLLIHYTSTLQSGIPSRFSGSGSGRDYSFSISNLEPEDNATYYCLQYDNLLTFGAGTKLELK

SEQ ID NO: 163 - protein, 7 aa, Artificial Sequence
  source: /note="Description of Artificial Sequence: Synthetic peptide"
GFSLTDY

SEQ ID NO: 164 - protein, 5 aa, Artificial Sequence
  source: /note="Description of Artificial Sequence: Synthetic peptide"
WNDGS

SEQ ID NO: 165 - protein, 10 aa, Artificial Sequence
  source: /note="Description of Artificial Sequence: Synthetic peptide"
NWYGGYWFAY

SEQ ID NO: 166 - protein, 11 aa, Artificial Sequence
  source: /note="Description of Artificial Sequence: Synthetic peptide"
RSSENIYSYLA

SEQ ID NO: 167 - protein, 7 aa, Artificial Sequence
  source: /note="Description of Artificial Sequence: Synthetic peptide"
NANALAE

SEQ ID NO: 168 - protein, 9 aa, Artificial Sequence
  source: /note="Description of Artificial Sequence: Synthetic peptide"
QHHYGTPFT

SEQ ID NO: 169 - protein, 5 aa, Artificial Sequence
  source: /note="Description of Artificial Sequence: Synthetic peptide"
DYDVH

SEQ ID NO: 170 - protein, 16 aa, Artificial Sequence
  source: /note="Description of Artificial Sequence: Synthetic peptide"
VIWNDGSTDYNTAFIS

SEQ ID NO: 171 - protein, 118 aa, Artificial Sequence
  source: /note="Description of Artificial Sequence: Synthetic polypeptide"
QAHLKESGPGLVAPSQSLSITCTVSGFSLTDYDVHWVRQSPGKGLEWLGVIWNDGSTDYNTAFISRLTISKDNSKSQVFFKMNSLQADDTAIYYCARNWYGGYWFAYWGQGTLVTVSA

SEQ ID NO: 172 - protein, 107 aa, Artificial Sequence
  source: /note="Description of Artificial Sequence: Synthetic polypeptide"
DIQMTQSPASLSASAGETVTITCRSSENIYSYLAWYQQKQGKSPQLLVYNANALAEGVPSRFSGSGSVTQFSLKINSLQPEDFGSYYCQHHYGTPFTFGSGTKLEIK

SEQ ID NO: 173 - DNA, 354 bp, Artificial Sequence
  source: /note="Description of Artificial Sequence: Synthetic polynucleotide"
caggtgcagctgaaggagtcaggacctggcctggtggcgccctcacagagcctgtccatcacctgcacagtctctggtttctcattaaccatctatgatgtacactgggttcgccagtctccaggaaagggtctggagtggctgggagtgatatggagtgatggaagcacagactataatgcagctttcatatctagactgagcatcagcaaggacaactccaagagccaagttttctttaaaatgaacagtctgcaagctgatgacacagccatatactactgtgccagaaattgggtcgaccaggcctggtttgcttactggggccaagggactctggtcactgtctctgca

SEQ ID NO: 174 - DNA, 321 bp, Artificial Sequence
  source: /note="Description of Artificial Sequence: Synthetic polynucleotide"
gacatccagatgactcagtctccagcctccctatctgcatctgtgggagaaactatcaccatcacatgtcgagcaagtaagaatatttacagttatttagcatggtatcagcagaaacagggaaaatctcctcagctcctggtctataatgcaaaaaccttaccagaaggtgtgccatcaaggttcagtggcagtggatcaggcacacagttttctctgaagatcaacagcctgcagcctgaagattttgggagttattactgtcaacatcattatggtactccgctcacgttcggtgctgggaccaagctggagctgaaa

SEQ ID NO: 175 - DNA, 363 bp, Artificial Sequence
  source: /note="Description of Artificial Sequence: Synthetic polynucleotide"
caggtccaactgcagcagtctggacctgagctggtgaagcctggagcttcagtgaagctgtcctgcaaggctgctggctacatcttcactgactatactataaactgggtgaagcagagtcctggacagggacttgagtggattggatggatttatcctggaagtggtaatcgtaaatacaatgacaagttcaagggcaaggccacaatgactgcagacaaatcctccagcacagcctacatgcagctcagcagcctgacctctgaggattctgcggtctatttctgtgcaagagagagtaactacgtggggtactatgctatggactattggggtcaaggaacctcagtcaccgtctcctca

SEQ ID NO: 176 - DNA, 336 bp, Artificial Sequence
  source: /note="Description of Artificial Sequence: Synthetic polynucleotide"
gatgttttgatgacccaaactccactctccctgcctgtcagtcttggagatcaagcctccatctcttgcagatctagtcagagcgttgtaaatagtaatggaaacacctatttagaatggtacctgcagaaaccaggccagtctccaaatctcctgatctacaaagtttccaatcgattttctggggtcccagacaggttcagtggcagtggatcggggacagatttcacactcaagatcagcagagtggaggctgaggatctgggagtttattactgttttcaaggttcacatgttccgtggacgttcggtggaggcaccaagctggaaatcaaa

SEQ ID NO: 177 - DNA, 363 bp, Artificial Sequence
  source: /note="Description of Artificial Sequence: Synthetic polynucleotide"
caggtccagctgcagcagtctggagctgagctggtaaggcctgggacttcagtgaagatgtcctgcaaggctgctggatacaccttcacaaactactggataggttgggtaaagcagaggcctggacatggccttgagtggattggagatatttaccctggaggtataggaggtggttatactaagtacaatgagaagttcaagggcaaggccacactgactgcagacacatcctccagcacagcctacatgcagctcggcagcctgacatctgaggactctgccatctatttctgttcaagatcggaaactggacgggctatggactactggggtcaaggaacctcagtcaccgtctcctca

SEQ ID NO: 178 - DNA, 318 bp, Artificial Sequence
  source: /note="Description of Artificial Sequence: Synthetic polynucleotide"
gacatccagatgacacagtctccatcctcactgtctgcatctctgggaggcaaagtcaccatcacttgcaaggcaagccaagacattaataagtatatagcttggtaccaacacaagcctggaaaaggtcctaggctgctcatacattacacatctacattaaagccaggcatcccatcaaggttcagtggaagtgggtctgggagagattattccttcagcatcagtgacctggagcctgaagatattgcaacttattattgtctacagtatgataatctgaacacgttcggaggggggaccaagctggaaataaaa

SEQ ID NO: 179 - DNA, 360 bp, Artificial Sequence
  source: /note="Description of Artificial Sequence: Synthetic polynucleotide"
gagatccagctgcagcagtctggacctgagctggtgaagcctggggcttcagtgaaggtgtcctgcaaggcttctggttattcattcactgactacaacatctactgggtgaagcagagccatggaaagagccttgagtggattggatatattgatccttccaatggtggtcctggctacaaccagaagttcaggggcaaggccacattgactgttgacaagtcctccagcacagccttcctgcatctcaacagcctgacatctgaggactctgcagtctattactgtgcaagaagggacaactacggctcggggactatggactactggggtcaaggaacctcagtcaccgtctcctca

SEQ ID NO: 180 - DNA, 321 bp, Artificial Sequence
  source: /note="Description of Artificial Sequence: Synthetic polynucleotide"
gacattgtgatgacccagtctcaaaaattcatgtccacatcagtaggagacagggtcagcatcacctgtaaggccagtcagaatgtgggtactgatgtatcctggtatcaacagaaaccagggaaatctcctaaaccactgatttactgggcatcaaaccggttcactggagtccctgatcgcttcataggtagtggatctgggacagatttcactctcaccatcagcaatgtgcagtctgaagacttggcagattatttctgtgagcaatatagcatctatccgctcacgttcggtgctgggaccaagctggagctgaaa

SEQ ID NO: 181 - DNA, 360 bp, Artificial Sequence
  source: /note="Description of Artificial Sequence: Synthetic polynucleotide"
gagatccagctgcagcagtctggacctgagctggtgaagcctggggcgtcagtgaaggtatcctgcaaggcttctggttactcattcactgacgacaacatgtactgggtgaagcagagccatggaaagagccttgagtggattggatatattgatcctctcaatggtggtactggctacaaccagaaattcaagggcaaggccacactgactgttgacaagtcctccagcacagccttcctgcatctcaacagcctgacatctgaggactctgcagtctattactgtgcaagaagggacaactacgccacggggactatggactactggggtcaaggaacctcagtcaccgtctcctca

SEQ ID NO: 182 - DNA, 321 bp, Artificial Sequence
  source: /note="Description of Artificial Sequence: Synthetic polynucleotide"
gacattgtgatgacccagtctcaaaaattcatgtccacatcagtaggagacagggtcagcatcacctgcaaggccagtaagaatgtgggtactgatgtatcctggtatcaacagaaaccagggaaatctcctaaaccactgatttactgggcatcaaaccggttcactggagtccctgatcgcttcacaggcagtggatctgggacagatttcactctcaccatcaacaatgtgcagtctgaagacttggcagattatttctgtgagcaatatagcagctatccgctcacgttcggtgctgggaccaagctggagctgaaa

SEQ ID NO: 183 - DNA, 360 bp, Artificial Sequence
  source: /note="Description of Artificial Sequence: Synthetic polynucleotide"
gaggtccagctgcagcagtctggccctgagctggtgaagcctggggcttcagtgaagatatcctgcaaggcttctggatacacattcactgactacaacatggactgggtgaagcagagccatggaaagagccttgagtggattggaaatatttatcctatcaatggttatactggctacaaccagaggttcaagaacaaggccacattgactgtagacaagtcctccagcacagcctacatggaactccacagcctgacatctgaggactctgcggtctattactgcgcaagagatagtaactacgttggctggtacttcgatgtctggggcgcagggaccacggtcaccgtctcctca

SEQ ID NO: 184 - DNA, 336 bp, Artificial Sequence
  source: /note="Description of Artificial Sequence: Synthetic polynucleotide"
gatgttgtgatgacccaaactccactctccctgcctgtcagtcttggagatcaagcctccatctcttgcagatctagtcagagccttgtacacagtaatggaaacacctatttacattggtacctgcagaagccaggccagtctccaaagctcctgatctacaaagtttccaaccgattttctggggtcccagacaggttcagtggcagtggatcagggacagatttcacattcaagatcagcagagtggaggctgaggatctgggagtttatttctgctctcaaagtacacatgttcctcggacgttcggtggaggcaccaagctggaaatcaaa

SEQ ID NO: 185 - DNA, 333 bp, Artificial Sequence
  source: /note="Description of Artificial Sequence: Synthetic polynucleotide"
gacattgtgctgacacagtctcctgcttccttaactgtatctctggggcagagggccaccttctcatgcagggccagcaaaagtgtcagtacatctggctatagttatatgcactggtaccaacagaaaccaggacagccacccaaactcctcatctattttacatccgacctagaacctggggtccctgccaggttcactggcagtgggtctgggacagacttcaccctcaacatccatcctgtggaggaggaggatgctgcaacctattactgtcagcacagtagggagcttccgtaccccttcggaggggggaccaagttggaaataaaa

SEQ ID NO: 186 - DNA, 354 bp, Artificial Sequence
  source: /note="Description of Artificial Sequence: Synthetic polynucleotide"
caggtccagctacagcagtctggacctgagctggtgaagcctggggcttcagtgaagatatcctgcaaggcttctggctacaccttcgctgactactatataaactgggtgaagcagaggcctggacagggacttgagtggattggatggatttttcctggaagtggtagtacttactacaatgagaagttcaagggcaaggccacacttactgtagacaaatcctccagcacagcctacatgttgctcagcagcctgacctctgaggactctgcggtctatttctgtgcaagaggggactccggtagggctatggactactggggtcaaggaacctcagtcaccgtctcctca

SEQ ID NO: 187 - DNA, 318 bp, Artificial Sequence
  source: /note="Description of Artificial Sequence: Synthetic polynucleotide"
gacatccagatgacacagtctccatcctcactgtctgcatctctgggaggcaaagtcaccatcacttgcaaggcaagccaagacattaacaaatatatagcttggtaccaacacaagcctggaaaaggtcctaggctgctcatacattacacatctacattacagtcaggcatcccatcaaggttcagtggaagtgggtctgggagagattattccttcagcatcagcaacctggagcctgaagataatgcaacttattattgtctacagtatgataatcttctcacgttcggtgctgggaccaagctggagctgaaa

SEQ ID NO: 188 - DNA, 354 bp, Artificial Sequence
  source: /note="Description of Artificial Sequence: Synthetic polynucleotide"
caggcgcacctgaaggagtcaggacctggcctggtggcgccctcacagagcctgtccatcacctgcacagtctctggtttctcattaaccgactatgatgtacactgggttcgccagtctccaggaaagggtctggagtggctgggagtgatatggaatgatggaagcacagactataatacagctttcatatctagactgaccatcagcaaggacaactccaagagccaagttttctttaaaatgaacagtctgcaagctgatgacacagccatatactactgtgccagaaattggtatggtggctactggtttgcttactggggccaagggactctggtcactgtctctgca

SEQ ID NO: 189 - DNA, 321 bp, Artificial Sequence
  source: /note="Description of Artificial Sequence: Synthetic polynucleotide"
gacatccagatgactcagtctccagcctccctatctgcatctgcgggagaaactgtcaccatcacatgtcgatcaagtgagaatatttacagttatttagcatggtatcagcagaaacagggaaaatctcctcagctcctagtctataatgcaaatgccttagcagaaggtgtgccatcgaggttcagtggcagtggatcagtcacacagttttctctgaagatcaacagcctgcagcctgaagattttgggagttattactgtcaacatcattatggtactccattcacgttcggctcggggacaaagttggaaataaaa

SEQ ID NO: 190 - protein, 120 aa, Artificial Sequence
  source: /note="Description of Artificial Sequence: Synthetic polypeptide"
QVQLQESGPGLVKPSQTLSLTCTVSGYSITSGYYWNWIRQHPGKGLEWIGYISYDGYNNYNPSLKNRVTISVDTSKNQFSLKLSSVTAADTAVYYCARYYDYEDWYFGVWGQGTMVTVSS

SEQ ID NO: 191 - protein, 120 aa, Artificial Sequence
  source: /note="Description of Artificial Sequence: Synthetic polypeptide"
QVQLQESGPGLVKPSQTLSLTCTVSGYSITSGYYWSWIRQHPGKGLEWIGYISYDGYTYYNPSLKSRVTISVDTSKNQFSLKLSSVTAADTAVYYCARYYDYEDWYFGVWGQGTMVTVSS

SEQ ID NO: 192 - protein, 120 aa, Artificial Sequence
  source: /note="Description of Artificial Sequence: Synthetic polypeptide"
QVQLQESGPGLVKPSQTLSLTCTVSGYSITSGYYWNWIRQHPGKGLEWIGYISYDGYNNYNPSLKSRVTISRDTSKNQFSLKLSSVTAADTAVYYCARYYDYEDWYFGVWGQGTMVTVSS

SEQ ID NO: 193 - protein, 120 aa, Artificial Sequence
  source: /note="Description of Artificial Sequence: Synthetic polypeptide"
QVQLQQWGAGLLKPSETLSLTCAVYGYSITSGYYWNWIRQPPGKGLEWIGYISYDGYNNYNPSLKNRVTISVDTSKNQFSLKLSSVTAADTAVYYCANYYDYEDWYFGVWGQGTTVTVSS

SEQ ID NO: 194 - protein, 120 aa, Artificial Sequence
  source: /note="Description of Artificial Sequence: Synthetic polypeptide"
QVQLQQWGAGLVKPSETLSLTCAVYGYSITSGYYWNWIRQPPGKGLEWIGYISYDGYNNYNPSLKNRVTISRDTSKNQFSLKLSSVTAADTAVYYCANYYDYEDWYFGVWGQGTTVTVSS

SEQ ID NO: 195 - protein, 120 aa, Artificial Sequence
  source: /note="Description of Artificial Sequence: Synthetic polypeptide"
QVQLQESGPGLVKPSETLSLTCTVSGYSITSGYYWNWIRQPPGKGLEWIGYISYDGYNNYNPSLKNRVTISVDTSKNQFSLKLSSVTAADTAVYYCANYYDYEDWYFGVWGQGTTVTVSS

SEQ ID NO: 196 - protein, 120 aa, Artificial Sequence
  source: /note="Description of Artificial Sequence: Synthetic polypeptide"
QVQLQESGPGLVKPSETLSLTCTVSGYSITSGYYWNWIRQPPGKGLEWIGYISYDGYNNYNPSLKNRVTISRDTSKNQFSLKLSSVTAADTAVYYCANYYDYEDWYFGVWGQGTTVTVSS

SEQ ID NO: 197 - protein, 120 aa, Artificial Sequence
  source: /note="Description of Artificial Sequence: Synthetic polypeptide"
QVQLQESGPGLMKPSETLSLTCSVSGYSITSGYYWSWIRKPPGKGLEYIGYVSYDGSTYYNPSLKSRVTISVDTSKNRFSLKLNSVTAADTAVYYCANYYDYEDWYFGYWGQGILVTVSS

SEQ ID NO: 198 - protein, 120 aa, Artificial Sequence
  source: /note="Description of Artificial Sequence: Synthetic polypeptide"
QVQLQESGPGLMKPSETLSLTCSVSGYSITSGYYWNWIRKPPGKGLEWIGYISYDGYNNYNPSLKSRVTISRDTSKNRFSLKLNSVTAADTAVYYCANYYDYEDWYFGVWGQGILVTVSS

SEQ ID NO: 199 - protein, 120 aa, Artificial Sequence
  source: /note="Description of Artificial Sequence: Synthetic polypeptide"
EVQLVESGGGLVQPGGSLRLSCAVSGYSITSGYYWNWIRQAPGKGLEWVASISYDGYNNYNPSVKGRITISRDDSKNTFYLQMNSLRAEDTAVYYCANYYDYEDWYFGVWGQGTLVTVSS

SEQ ID NO: 200 - protein, 120 aa, Artificial Sequence
  source: /note="Description of Artificial Sequence: Synthetic polypeptide"
EVQLVESGGGLVQPGGSLRLSCAVSGYSITSGYYWNWIRQAPGKGLEWVAYISYDGYNNYNPSVKGRITISRDTSKNTFYLQMNSLRAEDTAVYYCANYYDYEDWYFGVWGQGTLVTVSS

SEQ ID NO: 201 - protein, 120 aa, Artificial Sequence
  source: /note="Description of Artificial Sequence: Synthetic polypeptide"
QVQLVESGGGVVQPGRSLRLSCAASGYSITSGYYWNWVRQAPGKGLEWVAYISYDGYNNYNPSVKGRFTISRDNSKNTLYLQMNSLRAEDTAVYYCANYYDYEDWYFGVWGQGTMVTVSS

SEQ ID NO: 202 - protein, 111 aa, Artificial Sequence
  source: /note="Description of Artificial Sequence: Synthetic polypeptide"
EIVLTQSPATLSLSPGERATLSCRASESVSIIGTNSIHWYQQKPGQAPRLLIYHASNLETGIPARFSGSGPGTDFTLTISSLEPEDFAVYYCLQSRKIPYTFGQGTKLEIK

SEQ ID NO: 203 - protein, 111 aa, Artificial Sequence
  source: /note="Description of Artificial Sequence: Synthetic polypeptide"
DIVLTQSPASLAVSPGQRATITCRASESVSIIGTNSIHWYQQKPGQPPKLLIYHASNLETGVPARFSGSGSGTDFTLTINPVEANDTANYYCLQSRKIPYTFGGGTKLEIK

SEQ ID NO: 204 - protein, 111 aa, Artificial Sequence
  source: /note="Description of Artificial Sequence: Synthetic polypeptide"
EIVMTQSPATLSVSPGERATLSCRASESVSIIGTNSLHWYQQKPGQAPRLLIYHASQSISGIPARFSGSGSGTEFTLTISSLQSEDFAVYYCQQSRKIPYTFGGGTKVEIK

SEQ ID NO: 205 - protein, 111 aa, Artificial Sequence
  source: /note="Description of Artificial Sequence: Synthetic polypeptide"
EIVMTQSPATLSVSPGERATLSCRASESVSIIGTNSIHWYQQKPGQAPRLLIYHASNLETGIPARFSGSGSRTEFTLTISSLQSEDFAVYYCLQSRKIPYTFGGGTKVEIK

SEQ ID NO: 206 - protein, 111 aa, Artificial Sequence
  source: /note="Description of Artificial Sequence: Synthetic polypeptide"
DIQLTQSPSSLSASVGDRVTITCRASESVSIIGTNSMNWYQQKPGKAPKLLIYHASYLESGVPSRFSGSGSGTDFTLTISSLQPEDFATYYCLQSRKIPYTFGQGTKVEIK

SEQ ID NO: 207 - protein, 111 aa, Artificial Sequence
  source: /note="Description of Artificial Sequence: Synthetic polypeptide"
DIQLTQSPSSLSASVGDRVTITCRASESVSIIGTNSMHWYQQKPGKAPKLLIYHASNLESGVPSRFSGSGSRTDFTLTISSLQPEDFATYYCLQSRKIPYTFGQGTKVEIK

SEQ ID NO: 208 - protein, 111 aa, Artificial Sequence
  source: /note="Description of Artificial Sequence: Synthetic polypeptide"
DIQMTQSPSSLSASVGDRVTITCRASESVSIIGTNSMHWYQQKPGKAPKLLIYHASNLESGVPSRFSGSGSGTDFTFTISSLQPEDIATYYCLQSRKIPYTFGQGTKVEIK

SEQ ID NO: 209 - protein, 120 aa, Artificial Sequence
  source: /note="Description of Artificial Sequence: Synthetic polypeptide"
QVQLVQSGAEVKKPGASVKVSCKASGYTFTDYTIHWVRQAPGQGLEWMGWIYPLRGSINYNEKFKDRVTSTRDTSISTAYMELSRLRSDDTVVYYCARHGAYYSNAFDYWGQGTLVTVSS

SEQ ID NO: 210 - protein, 120 aa, Artificial Sequence
  source: /note="Description of Artificial Sequence: Synthetic polypeptide"
QVQLVQSGAEVKKPGASVKVSCKASGYTFTDYYMHWVRQAPGQGLEWMGRIYPLRGSTNYAQKFQGRVTSTRDTSISTAYMELSRLRSDDTVVYYCARHGAYYSNAFDYWGQGTLVTVSS

SEQ ID NO: 211 - protein, 120 aa, Artificial Sequence
  source: /note="Description of Artificial Sequence: Synthetic polypeptide"
QVQLVQSGAEVKKPGASVKVSCKASGYTFTDYTIHWVRQAPGQGLEWMGWIYPLRGSINYNEKFKDRVTMTADTSSSTAYMELSRLRSDDTVVYYCARHGAYYSNAFDYWGQGTLVTVSS

SEQ ID NO: 212 - protein, 120 aa, Artificial Sequence
  source: /note="Description of Artificial Sequence: Synthetic polypeptide"
QVQLVQSGAEVKKPGASVKVSCEASGYTFTDYTIHWVRQAPGKGLEWMGWIYPLRGSINYNEKFKDRVTMTADTSTDTAYMELSSLRSKDTAVYYCARHGAYYSNAFDYWGQGTLVTVSS

SEQ ID NO: 213 - protein, 120 aa, Artificial Sequence
  source: /note="Description of Artificial Sequence: Synthetic polypeptide"
QVQLVQSGAEVVKPGASVKLSCKASGYTFTDYTMYWVKQAPGQGLEWIGEIYPLRGSINFNEKFKSKATLTVDKSASTAYMELSSLRSEDTAVYYCARHGAYYSNAFDYWGQGTLVTVSS

SEQ ID NO: 214 - protein, 120 aa, Artificial Sequence
  source: /note="Description of Artificial Sequence: Synthetic polypeptide"
QVQLVQSGAEVVKPGASVKLSCKASGYTFTDYTMHWVKQAPGQGLEWIGEIYPLRGSINFNEKFKSKATLTVDKSASTAYMELSSLRSEDTAVYYCARHGAYYSNAFDYWGQGTLVTVSS

SEQ ID NO: 215 - protein, 111 aa, Artificial Sequence
  source: /note="Description of Artificial Sequence: Synthetic polypeptide"
EIVLTQSPATLSLSPGERATLSCRASESVDNDGIRFMHWYQQKPGQAPRLLIYRASNLESGIPARFSGSGPGTDFTLTISSLEPEDFAVYYCQQSNKDPYTFGQGTKLEIK

SEQ ID NO: 216 - protein, 111 aa, Artificial Sequence
  source: /note="Description of Artificial Sequence: Synthetic polypeptide"
EIVLTQSPATLSLSPGERATLSCRASESVDNDGIRFMHWYQQKPGQAPRLLIYRASNLESGIPARFSGSGPGTDFTLTISSLEPEDVAVYYCQQSNKDPYTFGQGTKLEIK

SEQ ID NO: 217 - protein, 111 aa, Artificial Sequence
  source: /note="Description of Artificial Sequence: Synthetic polypeptide"
DIVMTQSPASLAVSLGERATINCRASESVDNDGIRFMHWYQQKPGQPPKLLIYRASNLESGVPDRFSGSGSRTDFTLTISSLQAEDVAVYYCQQSNKDPYTFGGGTKVEIK

SEQ ID NO: 218 - protein, 111 aa, Artificial Sequence
  source: /note="Description of Artificial Sequence: Synthetic polypeptide"
DIVMTQSPASLAVSLGERATINCRASESVDNDGIRFMHWYQQKPGQPPKLLIYRASNLESGVPDRFSGSGSRTDFTLTINSLQAEDVAVYYCQQSNKDPYTFGGGTKVELK

SEQ ID NO: 219 - protein, 111 aa, Artificial Sequence
  source: /note="Description of Artificial Sequence: Synthetic polypeptide"
DIVLTQSPATLSVSPGERATISCRASESVDNDGIRFMHWYQQKPGQPPKLLIYRASNLESGVPARFSGSGSRTDFTLTISSVEPEDFATYYCQHSWEIPPTFGGGTKLEIK

SEQ ID NO: 220 - protein, 118 aa, Artificial Sequence
  source: /note="Description of Artificial Sequence: Synthetic polypeptide"
QVQLVESGGGVVQPGRSLRLSCAASGFSLTIYDVHWVRQAPGKGLEWVAVIWSDGSTDYNAAFISRFTISRDNSKNTLYLQMNSLRAEDTAVYYCARNWVDQAWFAYWGQGTLVTVSS

SEQ ID NO: 221 - protein, 118 aa, Artificial Sequence
  source: /note="Description of Artificial Sequence: Synthetic polypeptide"
QVQLVESGGGVVQPGRSLRLSCAASGFSLTIYDVHWVRQAPGKGLEWVGVIWSDGSTDYNAAFISRFTISKDNSKNTLYLQMNSLRAEDTAVYYCARNWVDQAWFAYWGQGTLVTVSS

SEQ ID NO: 222 - protein, 118 aa, Artificial Sequence
  source: /note="Description of Artificial Sequence: Synthetic polypeptide"
QVQLVESGGGVVQPGRSLRLSCAASGFSLTIYDVHWVRQAPGKGLEWVAVIWSDGSTDYADSVKGRFTISKDNSKNTLYLQMNSLRAEDTAVYYCARNWVDQAWFAYWGQGTLVTVSS

SEQ ID NO: 223 - protein, 118 aa, Artificial Sequence
  source: /note="Description of Artificial Sequence: Synthetic polypeptide"
QVQLVESGGGVVQPGRSLRLSCAVSGFSLTIYDVHWVRQAPGKGLEWVGVIWSDGSTDYADSVKGRFTISKDNSKNTVYLQMNSLRAEDTAVYYCARNWVDQAWFAYWGQGTLVTVSS

SEQ ID NO: 224 - protein, 118 aa, Artificial Sequence
  source: /note="Description of Artificial Sequence: Synthetic polypeptide"
QVQLQESGPGLVKPSETLSLTCTVSGFSLTIYDVHWIRQPPGKGLEWIGVIWSDGSTDYNAAFISRVTISVDTSKNQFSLKLSSVTAADTAVYYCARNWVDQAWFAYWGQGTLVTVSS

SEQ ID NO: 225 - protein, 118 aa, Artificial Sequence
  source: /note="Description of Artificial Sequence: Synthetic polypeptide"
QVQLQESGPGLVKPSETLSLTCTVSGFSLTIYDVHWVRQPPGKGLEWIGVIWSDGSTDYNPSLKSRVTISKDTSKNQVSLKLSSVTAADTAVYYCARNWVDQAWFAYWGQGTLVTVSS

SEQ ID NO: 226 - protein, 118 aa, Artificial Sequence
  source: /note="Description of Artificial Sequence: Synthetic polypeptide"
QVQLQESGPGLMKPSETLSLTCSVSGDSITIYDWHWIRQPPGKGLEWIGVVWSDGSTDYNPSLKSRVTISVDTSKNRFSLKLSSVTAADTAVYYCARNWVDQAWFAYWGQGTLVTVSS

SEQ ID NO: 227 - protein, 118 aa, Artificial Sequence
  source: /note="Description of Artificial Sequence: Synthetic polypeptide"
QVQLQESGPGLVKPSETLSLTCTVSGFSLTIYDVHWIRQPPGKGLEWIGVIWSDGSTDYNPSLKSRVTISKDNSKNQFSLKLSSVTAADTAVYYCARNWVDQAWFAYWGQGTLVTVSS

SEQ ID NO: 228 - protein, 107 aa, Artificial Sequence
  source: /note="Description of Artificial Sequence: Synthetic polypeptide"
DIQMTQSPSSLSASVGDRVTITCRASKNIYSYLAWYQQKPGKAPKLLIYNAKTLPEGVPSRFSGSGSGTDFTLTISSLQPEDFATYYCQHHYGTPLTFGQGTKLEIK

SEQ ID NO: 229 - protein, 107 aa, Artificial Sequence
  source: /note="Description of Artificial Sequence: Synthetic polypeptide"
DIQMTQSPSSLSASVGDRVTITCRASKNIYSYLAWYQQKPGKAPKLLVYNAKTLPEGVPSRFSGSGSGTDFTLTISSLQPEDFATYYCQHHYGTPLTFGQGTKLEIK

SEQ ID NO: 230 - protein, 107 aa, Artificial Sequence
  source: /note="Description of Artificial Sequence: Synthetic polypeptide"
EIVLTQSPATLSLSPGERATLSCRASKNIYSYLAWYQQKPGQAPRLLIYNAKTRATGIPARFSGSGSGTDFTLTISSLEPEDFAVYYCQHHYGTPLTFGQGTKLEIK

SEQ ID NO: 231 - protein, 107 aa, Artificial Sequence
  source: /note="Description of Artificial Sequence: Synthetic polypeptide"
EIVLTQSPATLSLSPGERATLSCRASKNIYSYLAWYQQKPGQAPRLLVYNAKTLPEGIPARFSGSGSGTDFTLTISSLEPEDFAVYYCQHHYGTPLTFGQGTKLEIK

SEQ ID NO: 232 - protein, 107 aa, Artificial Sequence
  source: /note="Description of Artificial Sequence: Synthetic polypeptide"
EIVMTQSPATLSVSPGERATLSCRASKNIYSYLAWYQQKPGQAPRLLIYNAKTRATGIPARFSGSGSGTEFTLTISSLQSEDFAVYYCQHHYGTPLTFGGGTKVEIK

SEQ ID NO: 233 - protein, 107 aa, Artificial Sequence
  source: /note="Description of Artificial Sequence: Synthetic polypeptide"
DIQLTQSPSFLSASVGDRVTITCRASKNIYSYLAWYQQKPGKAPKLLIYNAKSLQSGVPSRFSGSGSGTEFTLTISSLQPEDFATYYCQHHYGTPLTFGGGTKLEIK

SEQ ID NO: 234 - protein, 107 aa, Artificial Sequence; identical to SEQ ID NO: 233
  source: /note="Description of Artificial Sequence: Synthetic polypeptide"

SEQ ID NO: 235 - protein, 118 aa, Artificial Sequence
  source: /note="Description of Artificial Sequence: Synthetic polypeptide"
QLQLQESGSGLVKPSQTLSLTCAVSGFSLTDYDVHWVRQPPGKGLEWIGVIWNDGSTDYNPSLISRVTISKDNSKNQVSLKLSSVTAADTAVYYCARNWYGGYWFAYWGQGTLVTVSS

SEQ ID NO: 236 - protein, 118 aa, Artificial Sequence
  source: /note="Description of Artificial Sequence: Synthetic polypeptide"
QLQLQESGSGLVKPSQTLSLTCAVSGGSITDYDWHWVRQPPGKGLEWIGVIWNDGSTDYNPSLISRVTISVDNSKNQFSLKLSSVTAADTAVYYCARNWYGGYWFAYWGQGTLVTVSS

SEQ ID NO: 237 - protein, 118 aa, Artificial Sequence
  source: /note="Description of Artificial Sequence: Synthetic polypeptide"
QVQLVESGGGVVQPGRSLRLSCAASGFSFTDYDMHWVRQAPGKGLEWVAVIWNDGSTDYATSVIGRFTISRDNSKNTLYLQMNSLRAEDTAVYYCARNWYGGYWFAYWGQGTLVTVSS

SEQ ID NO: 238 - protein, 118 aa, Artificial Sequence
  source: /note="Description of Artificial Sequence: Synthetic polypeptide"
QVQLVESGGGVVQPGRSLRLSCAASGFSFTDYDMHWVRQAPGKGLEWVGVIWNDGSTDYATSVIGRFTISRDNSKNTLYLQMNSLRAEDTAVYYCARNWYGGYWFAYWGQGTLVTVSS

SEQ ID NO: 239 - protein, 118 aa, Artificial Sequence
  source: /note="Description of Artificial Sequence: Synthetic polypeptide"
QVQLQESGPGLMKPSETLSLTCSVSGGSITDYDWHWIRQPPGKGLEWIGVVWNDGSTDYNPSLKSRVTISVDTSKNRFSLKLNSVTAADTAVYYCARNWYGGYWFAYWGQGILVTVSS

SEQ ID NO: 240 - protein, 118 aa, Artificial Sequence
  source: /note="Description of Artificial Sequence: Synthetic polypeptide"
QVTLKESGPALVKPTQTLTLTCTFSGFSLTDYDVHWIRQPPGKALEWLAVIWNDGSTDYSPSLKSRLTITKDTSKNQVVLTMTNMDPVDTATYYCARNWYGGYWFAYWGQGTLVTVSS

SEQ ID NO: 241 - protein, 107 aa, Artificial Sequence
  source: /note="Description of Artificial Sequence: Synthetic polypeptide"
DIQMTQSPSSLSASVGDRVTITCRSSENIYSYLAWYQQKPGKAPKLLVYNANALAEGVPSRFSGSGSVTDFTLTISSLQPEDFATYYCQHHYGTPFTFGQGTKLEIK

SEQ ID NO: 242 - protein, 107 aa, Artificial Sequence
  source: /note="Description of Artificial Sequence: Synthetic polypeptide"
DIQMTQSPSTLSASVGDRVTITCRSSENIYSYLAWYQQKPGKAPKLLVYNANALAEGVPSRFSGSGSVTEFTLTISSLQPDDFATYYCQHHYGTPFTFGQGTKLEIK

SEQ ID NO: 243 - protein, 107 aa, Artificial Sequence
  source: /note="Description of Artificial Sequence: Synthetic polypeptide"
EIVMTQSPATLSVSPGERATLSCRASENIYSYLAWYQQKPGQAPRLLIYNANASAEGIPARFSGSGSGTEFTLTISSLQSEDFAVYYCQQHYGTPFTFGGGTKVEIK

SEQ ID NO: 244 - protein, 107 aa, Artificial Sequence
  source: /note="Description of Artificial Sequence: Synthetic polypeptide"
DIQMTQSPSSLSASVGDRVTITCRASENIYSYLAWYQQKPGKAPKLLLYNANRLESGVPSRFSGSGSGTDFTLTISSLQPEDFASYYCQHHYGTPFTFGSGTKLEIK

SEQ ID NO: 245 - protein, 107 aa, Artificial Sequence
  source: /note="Description of Artificial Sequence: Synthetic polypeptide"
DIQMTQSPSSLSASVGDRVTITCRASENIYSYLAWYQQKPGKAPKLLLYNANRLESGVPSRFSGSGSGTDYTLTISSLQPEDFASYYCQHHYGTPFTFGSGTKLEIK

SEQ ID NO: 246 - protein, 121 aa, Artificial Sequence
  source: /note="Description of Artificial Sequence: Synthetic polypeptide"
QVQLVQSGAEVKKPGASVKVSCKASGYTFTNYWIGWVRQAPGQGLEWMGDIYPGGIGGGYTKYNEKFKGRVTMTADTSTSTAYMELRSLRSDDTAVYYCSRSETGRAMDYWGQGTLVTVSS

SEQ ID NO: 247 - protein, 121 aa, Artificial Sequence
  source: /note="Description of Artificial Sequence: Synthetic polypeptide"
QVQLVQSGAEVKKPGASVKVSCKASGYTFTNYWIGWVRQAPGQGLEWMGDIYPGGIGGGYTKYAQKLQGRVTMTADTSTSTAYMELRSLRSDDTAVYYCSRSETGRAMDYWGQGTLVTVSS

SEQ ID NO: 248 - protein, 121 aa, Artificial Sequence
  source: /note="Description of Artificial Sequence: Synthetic polypeptide"
QVQLVQSGAEVKKPGASVKVSCKASGYTFTNYWIGWVRQAPGQGLEWMGDIYPGGIGGGYTKYAQKFQGRVTMTADTSTSTAYMELSSLRSEDTAVYYCSRSETGRAMDYWGQGTLVTVSS

SEQ ID NO: 249 - protein, 121 aa, Artificial Sequence
  source: /note="Description of Artificial Sequence: Synthetic polypeptide"
QVQLVQSGAEVKKPGASVKVSCKASGYTFTNYWIGWVRQAPGQGLEWMGDIYPGGIGGGYTKYNEKFKGRVTMTADTSTSTAYMELSSLRSEDTAVYFCSRSETGRAMDYWGQGTLVTVSS

SEQ ID NO: 250 - protein, 121 aa, Artificial Sequence
  source: /note="Description of Artificial Sequence: Synthetic polypeptide"
QVQLVQSGAELKRPGASVKVSCKASGYTFTNYWMGWVKQAPGQGLEWMGDIYPGGIGGGYTNYAQKFKGKATMTADTSSSTAYMQLSRLRSEDTAVYYCSRSETGRAMDYWGQGTLVTVSS

SEQ ID NO: 251 - protein, 106 aa, Artificial Sequence
  source: /note="Description of Artificial Sequence: Synthetic polypeptide"
DIQMTQSPSSLSASVGDRVTITCQASQDINKYLAWYQQKPGKAPKLLIHYTSTLKPGVPSRFSGSGSGTDFTFTISSLQPEDIATYYCLQYDNLNTFGGGTKLEIK

SEQ ID NO: 252 - protein, 106 aa, Artificial Sequence
  source: /note="Description of Artificial Sequence: Synthetic polypeptide"
DIQMTQSPSSLSASVGDRVTITCKASQDINKYIAWYQQKPGKAPKLLIHYTSTLKPGVPSRFSGSGSGRDYTFTISSLQPEDIATYYCLQYDNLNTFGGGTKLEIK

SEQ ID NO: 253 - protein, 106 aa, Artificial Sequence
  source: /note="Description of Artificial Sequence: Synthetic polypeptide"
DIQMTQSPSSLSASVGDRVTITCQASQDINKYLAWYQQKPGKAPKLLIYYTSTLETGVPSRFSGSGSGTDFTFSISSLQPEDIATYYCLQYDNLNTFGGGTKLEIK

SEQ ID NO: 254 - protein, 118 aa, Artificial Sequence
  source: /note="Description of Artificial Sequence: Synthetic polypeptide"
QVQLVQSGAEVKKPGASVKVSCKASGYTFADYYINWVRQAPGKGLEWMGWIFPGSGSTYYNEKFKGRVTMTVDKSTSTAYMELSSLRSEDTAVYFCARGDSGRAMDYWGQGTLVTVSS

SEQ ID NO: 255 - protein, 118 aa, Artificial Sequence
  source: /note="Description of Artificial Sequence: Synthetic polypeptide"
QVQLVQSGAEVKKPGASVKVSCKASGYTFADYYMNWVRQAPGQGLEWMGWIFPGSGSTYYAEKFKGRVTSTRDTSISTAYMELSRLRSDDTVVYYCARGDSGRAMDYWGQGTLVTVSS

SEQ ID NO: 256 - protein, 118 aa, Artificial Sequence
  source: /note="Description of Artificial Sequence: Synthetic polypeptide"
QVQLVQSGAEVKKPGASVKVSCKASGYTFADYYINWVRQAPGQGLEWMGWIFPGSGSTYYAQKLQGRVTMTTDTSTSTAYMELRSLRSDDTAVYYCARGDSGRAMDYWGQGTLVTVSS

SEQ ID NO: 257 - protein, 118 aa, Artificial Sequence
  source: /note="Description of Artificial Sequence: Synthetic polypeptide"
QVQLVQSGAEVKKPGASVKVSCKASGYTFADYYINWVRQAPGQGLEWMGWIFPGSGSTYYAQKLQGRVTMTVDKSSSTAYMELRSLRSDDTAVYYCARGDSGRAMDYWGQGTLVTVSS

SEQ ID NO: 258 - protein, 118 aa, Artificial Sequence
  source: /note="Description of Artificial Sequence: Synthetic polypeptide"
QVQLVQSGAELKKPGASVKVSCKASGYTFADYYMNWVRQAPGQGLEWMGWIFPGSGSTYYNQKFQGRVTMTVDKSSSTAYMELSRLRSDDTAVYYCARGDSGRAMDYWGQGTLVTVSS

SEQ ID NO: 259 - protein, 106 aa, Artificial Sequence
  source: /note="Description of Artificial Sequence: Synthetic polypeptide"
DIQMTQSPSSLSASVGDRVTITCKASQDINKYIAWYQQKPGKAPKLLIHYTSTLQSGVPSRFSGSGSGTDFTFTISSLQPEDIATYYCLQYDNLLTFGQGTKLEIK

SEQ ID NO: 260 - protein, 106 aa, Artificial Sequence
  source: /note="Description of Artificial Sequence: Synthetic polypeptide"
DIQMTQSPSSLSASVGDRVTITCKASQDINKYIAWYQHKPGKAPKLLIHYTSTLQSGVPSRFSGSGSGRDYTFTISSLQPEDIATYYCLQYDNLLTFGQGTKLEIK

SEQ ID NO: 261 - protein, 106 aa, Artificial Sequence
  source: /note="Description of Artificial Sequence: Synthetic polypeptide"
DIQMTQSPSSLSASVGDRVTITCQASQDINKYLAWYQHKPGKAPKLLIHYTSTLETGVPSRFSGSGSGTDFTFTISSLQPEDIATYYCLQYDNLLTFGGGTKVEIK

SEQ ID NO: 262 - protein, 118 aa, Artificial Sequence
  source: /note="Description of Artificial Sequence: Synthetic polypeptide"
QVQLQESGPGLVKPSETLSLTCTVSGFSLTIYDVHWIRQPPGKGLEWIGVIWSDGSTDYNPSLKSRVTISKDTSKNQVSLKLSSVTAADTAVYYCARNWVDQAWFAYWGQGTLVTVSS

SEQ ID NO: 263 - protein, 118 aa, Artificial Sequence
  source: /note="Description of Artificial Sequence: Synthetic polypeptide"
QVQLQESGPGLVKPSETLSLTCTVSGGSITIYDWHWVRQPPGKGLEWIGVIWSDGSTDYNPSLKSRVTISKDTSKNQFSLKLSSVTAADTAVYYCARNWVDQAWFAYWGQGTLVTVSS

SEQ ID NO: 264 - protein, 118 aa, Artificial Sequence
  source: /note="Description of Artificial Sequence: Synthetic polypeptide"
QVQLQESGPGLVKPSETLSLTCTVSGGSITIYDWHWVRQPPGKGLEWIGVIWSDGSTDYNPSLKSRVTISVDTSKNQFSLKLSSVTAADTAVYYCARNWVDQAWFAYWGQGTLVTVSS

SEQ ID NO: 265 - protein, 118 aa, Artificial Sequence
  source: /note="Description of Artificial Sequence: Synthetic polypeptide"
QVQLQESGPGLVKPSETLSLTCTVSGGSITIYDWHWIRQPPGKGLEWIGVIWSDGSTDYNPSLKSRVTISVDTSKNQFSLKLSSVTAADTAVYYCARNWVDQAWFAYWGQGTLVTVSS

SEQ ID NO: 266 - protein, 7 aa, Artificial Sequence
  source: /note="Description of Artificial Sequence: Synthetic peptide"
DYSFTGY

SEQ ID NO: 267 - protein, 6 aa, Artificial Sequence
  source: /note="Description of Artificial Sequence: Synthetic peptide"
HPYYGG

SEQ ID NO: 268 - protein, 10 aa, Artificial Sequence
  source: /note="Description of Artificial Sequence: Synthetic peptide"
ERSNFHALDY

SEQ ID NO: 269 - protein, 5 aa, Artificial Sequence
  source: /note="Description of Artificial Sequence: Synthetic peptide"
GYNMN

SEQ ID NO: 270 - protein, 17 aa, Artificial Sequence
  source: /note="Description of Artificial Sequence: Synthetic peptide"
NIHPYYGGTSFNQKFMG

SEQ ID NO: 271 - protein, 119 aa, Artificial Sequence
  source: /note="Description of Artificial Sequence: Synthetic polypeptide"
EIQLQQSGAELVKPGASVKISCKASDYSFTGYNMNWVMQSHGKSLEWIGNIHPYYGGTSFNQKFMGKATLTADKSSSTAYMQLNSLTSEDSAVYYCARERSNFHALDYWGQGTSVTVSS

SEQ ID NO: 272 - protein, 111 aa, Artificial Sequence; identical to SEQ ID NO: 153
  source: /note="Description of Artificial Sequence: Synthetic polypeptide"

SEQ ID NO: 273 - protein, 16 aa, Artificial Sequence
  source: /note="Description of Artificial Sequence: Synthetic peptide"
VIWSDGSTDYNPSLKS

SEQ ID NO: 274 - protein, 11 aa, Artificial Sequence
  source: /note="Description of Artificial Sequence: Synthetic peptide"
QASQDINKYLA

SEQ ID NO: 275 - protein, 7 aa, Artificial Sequence
  source: /note="Description of Artificial Sequence: Synthetic peptide"
YTSTLET

SEQ ID NO: 276 - protein, 5 aa, Artificial Sequence
  source: /note="Description of Artificial Sequence: Synthetic peptide"
DYYMN

SEQ ID NO: 277 - protein, 17 aa, Artificial Sequence
  source: /note="Description of Artificial Sequence: Synthetic peptide"
WIFPGSGSTYYNQKFQG

SEQ ID NO: 278 - protein, 17 aa, Artificial Sequence
  source: /note="Description of Artificial Sequence: Synthetic peptide"
WIFPGSGSTYYAQKLQG

SEQ ID NO: 279 - skipped

SEQ ID NO: 280 - protein, 15 aa, Artificial Sequence
  source: /note="Description of Artificial Sequence: Synthetic peptide"
RASESVDNDGIRFLH

SEQ ID NO: 281 - protein, 7 aa, Artificial Sequence
  source: /note="Description of Artificial Sequence: Synthetic peptide"
RASNRET

SEQ ID NO: 282 - protein, 17 aa, Artificial Sequence
  source: /note="Description of Artificial Sequence: Synthetic peptide"
WIYPLRGSINYAQKFQG

SEQ ID NO: 283 - protein, 120 aa, Artificial Sequence
  source: /note="Description of Artificial Sequence: Synthetic polypeptide"
QVQLVQSGAEVKKPGASVKVSCKASGYTFTDYTIHWVRQATGQGLEWMGWIYPLRGSINYAQKFQGRVTMTANKSISTVYMELSSLRSEDTAVYFCARHGAYYSNAFDYWGQGTLVTVSS

SEQ ID NO: 284 - protein, 111 aa, Artificial Sequence
  source: /note="Description of Artificial Sequence: Synthetic polypeptide"
EIVMTQSPATLSVSPGERATLSCRASESVDNDGIRFLHWYQQKPGQAPRLLIYRASNRETGIPARFSGSGSGTEFTLTISSLQSEDFAVYYCQQSNKDPYTFGGGTKVEIK

SEQ ID NO: 285 - protein, 7 aa, Artificial Sequence
  source: /note="Description of Artificial Sequence: Synthetic peptide"
RASTRAT

SEQ ID NO: 286 - protein, 111 aa, Artificial Sequence
  source: /note="Description of Artificial Sequence: Synthetic polypeptide"
EIVMTQSPATLSVSPGERATLSCRASESVDNDGIRFLHWYQQKPGQAPRLLIYRASTRATGIPARFSGSGSRTEFTLTISSLQSEDFAVYYCQQSNKDPYTFGGGTKVEIK

SEQ ID NO: 287 - protein, 17 aa, Artificial Sequence
  source: /note="Description of Artificial Sequence: Synthetic peptide"
WIYPLRGSINYSPSFQG

SEQ ID NO: 288 - protein, 120 aa, Artificial Sequence
  source: /note="Description of Artificial Sequence: Synthetic polypeptide"
EVQLVQSGAEVKKPGESLKISCKASGYTFTDYTIHWVRQMPGKGLEWMGWIYPLRGSINYSPSFQGQVTISADKSISTVYLQWSSLKASDTAMYFCARHGAYYSNAFDYWGQGTLVTVSS

SEQ ID NO: 289 - protein, 120 aa, Artificial Sequence
  source: /note="Description of Artificial Sequence: Synthetic polypeptide"
QVQLVQSGAEVKKPGSSVKVSCKASGYTFTDYTIHWVRQAPGQGLEWMGWIYPLRGSINYAQKFQGRVTITADKSTSTAYMELSSLRSEDTAVYFCARHGAYYSNAFDYWGQGTLVTVSS

SEQ ID NO: 290 - protein, 17 aa, Artificial Sequence
  source: /note="Description of Artificial Sequence: Synthetic peptide"
WIYPLRGSINYAEKFKG

SEQ ID NO: 291 - protein, 120 aa, Artificial Sequence
  source: /note="Description of Artificial Sequence: Synthetic polypeptide"
QVQLVQSGAEVKKPGSSVKVSCKASGYTFTDYTIHWVRQAPGQGLEWMGWIYPLRGSINYAEKFKGRVTLTADKSTSTVYMELSSLRSEDTAVYFCARHGAYYSNAFDYWGQGTLVTVSS

SEQ ID NO: 292 - protein, 120 aa, Artificial Sequence
  source: /note="Description of Artificial Sequence: Synthetic polypeptide"
QVQLVQSGAEVKKPGASVKVSCKASGYTFTDYTIHWVRQAPGQGLEWMGWIYPLRGSINYAQKFQGRVTMTADKSISTVYMELSRLRSDDTAVYYCARHGAYYSNAFDYWGQGTLVTVSS

SEQ ID NO: 293 - protein, 7 aa, Artificial Sequence
  source: /note="Description of Artificial Sequence: Synthetic peptide"
RASTLET

SEQ ID NO: 294 - protein, 120 aa, Artificial Sequence
  source: /note="Description of Artificial Sequence: Synthetic polypeptide"
QVQLVQSGAEVKKPGASVKVSCKASGYTFTDYTIHWVRQATGQGLEWMGWIYPLRGSINYAQKFQGRVTMTANKSSSTVYMELSSLRSEDTAVYFCARHGAYYSNAFDYWGQGTLVTVSS

SEQ ID NO: 295 - protein, 111 aa, Artificial Sequence
  source: /note="Description of Artificial Sequence: Synthetic polypeptide"
EIVMTQSPATLSVSPGERATLSCRASESVDNDGIRFLHWYQQKPGQAPRLLIYRASTLETGIPARFSGSGSGTEFTLTISSLQSEDFAVYYCQQSNKDPYTFGGGTKVEIK

SEQ ID NO: 296 - protein, 120 aa, Artificial Sequence
  source: /note="Description of Artificial Sequence: Synthetic polypeptide"
QVQLVQSGAEVKKPGASVKVSCKASGYTFTDYTIHWVRQATGQGLEWMGWIYPLRGSINYAQKFQGRVTMTADKSISTVYMELSSLRSEDTAVYFCARHGAYYSNAFDYWGQGTLVTVSS

SEQ ID NO: 297 - DNA, 357 bp, Artificial Sequence
  source: /note="Description of Artificial Sequence: Synthetic polynucleotide"
gagatccagctgcagcagtctggagctgaactggtgaagcctggggcttcagtgaagatatcctgcaaggcttctgattactcattcactggctacaacatgaactgggtgatgcagagccatggaaagagccttgagtggattggaaatattcatccttactatggtggtactagcttcaatcagaagttcatgggcaaggccacattgactgcagacaaatcttccagcacagcctacatgcagctcaacagcctgacatctgaagactctgcagtctattactgtgcaagagagagaagtaacttccatgctctggactactggggtcagggaacctcagtcaccgtctcctca

SEQ ID NO: 298 - DNA, 333 bp, Artificial Sequence; identical to SEQ ID NO: 185
  source: /note="Description of Artificial Sequence: Synthetic polynucleotide"

SEQ ID NO: 299 - DNA, 354 bp, Artificial Sequence
  source: /note="Description of Artificial Sequence: Synthetic polynucleotide"
caggtacaactccaggaatccgggcctgggctcgtcaaaccaagcgaaacactctctctcacctgcaccgtttctgggttttctcttactatctatgacgtacattgggtaaggcaaccacccgggaaggggctggagtggatcggtgtaatctggtcagatggatctacagactacaacccatcccttaaaagcagggtgaccatttctaaggacacttccaagaaccaagtatcccttaaattgtcctctgtaaccgcagcagacaccgcagtttactactgcgcacgaaattgggttgaccaagcatggtttgcatattggggacagggaactcttgtcactgtgtcttca

SEQ ID NO: 300 - DNA, 321 bp, Artificial Sequence
  source: /note="Description of Artificial Sequence: Synthetic polynucleotide"
gatattcaaatgacccaatccccctcatcactttcagcatctgtcggtgatcgggtcaccattacttgcagagccagtaagaatatctacagctacctggcttggtatcagcaaaaacctggtaaggcccctaaacttctcgtttacaatgctaagacccttcccgagggagttccttccaggttttccggtagcgggagtggaacagatttcaccttgactatttctagcttgcagcccgaggatttcgctacatactactgccagcatcactatggaacccccctgaccttcggtcagggaaccaagctcgagatcaaa

SEQ ID NO: 301 - DNA, 354 bp, Artificial Sequence
  source: /note="Description of Artificial Sequence: Synthetic polynucleotide"
caagtccagctcgtacagagcggggcagagctgaagaagcctggggcctccgtcaaggtctcctgtaaggcttctggttacacatttgccgactactacatgaactgggtacggcaagccccaggtcaagggctggaatggatgggatggatttttccagggagcggcagcacttactacaaccagaaatttcaaggtcgtgtgacaatgaccgtggataaaagcagctctacagcttacatggagctttcccgcttgaggtccgatgatactgccgtatattattgtgcccgtggtgactcaggtagggccatggactattggggacagggcaccctcgtgaccgtgtccagc

SEQ ID NO: 302 - DNA, 318 bp, Artificial Sequence
  source: /note="Description of Artificial Sequence: Synthetic polynucleotide"
gatatccagatgacacaatccccttcatccttgagcgcatcagttggcgacagggtcaccataacttgtcaggctagtcaggatattaacaagtacctggcttggtatcaacacaagcctggaaaggcccccaaattgctgattcactacacctctacattggaaactggcgtacccagtcgcttttctgggagtggaagcggaactgatttcactttcactatatccagtcttcagccagaagatatcgcaacttactattgtcttcagtatgataacttgcttactttcggaggagggaccaaagttgaaatcaag

SEQ ID NO: 303 - DNA, 354 bp, Artificial Sequence
  source: /note="Description of Artificial Sequence: Synthetic polynucleotide"
caggtgcagttggtccaatccggggctgaggtgaagaagcctggggcctctgttaaagttagttgcaaggcatcaggctacaccttcgctgactactacatcaactgggttagacaggcccccgggcaggggttggagtggatgggttggatttttccaggatcaggttcaacatattacgcacaaaaactgcaaggtagagtaaccatgacaactgatactagcacctccacagcctatatggaactccgctctctcaggagtgacgatacagccgtttattactgcgcccgtggggattcaggccgtgcaatggattactggggtcaagggaccctcgtgaccgtaagttca

SEQ ID NO: 304 - DNA, 360 bp, Artificial Sequence
  source: /note="Description of Artificial Sequence: Synthetic polynucleotide"
caagttcagttggtgcaaagcggggcagaagtgaagaaacctggtgcttctgtgaaagtttcctgcaaggccagcggctacacctttactgattacacaatacactgggtacggcaggcaactgggcaaggattggaatggatggggtggatatacccattgcgagggtctataaactacgcacagaaatttcaaggtcgagtaacaatgacagccaacaaatcaataagcaccgtttatatggaactctcatctctcaggagtgaggataccgccgtgtatttctgcgcacgacacggtgcatattactcaaacgctttcgactattggggccagggcacccttgtgactgttagtagc

SEQ ID NO: 305 - DNA, 333 bp, Artificial Sequence
  source: /note="Description of Artificial Sequence: Synthetic polynucleotide"
gagatagtaatgactcagtctcccgctacacttagtgtaagcccaggggagcgagcaaccctcagttgcagagcatctgagagtgttgataatgatggaatacgttttctccattggtatcaacaaaaaccagggcaggcccccagattgctgatctaccgtgcttccaatcgcgagactggcattcctgcacgtttcagcggcagcggctccggaaccgagtttacacttactattagctcactccagtctgaagacttcgctgtgtattactgtcagcaatccaacaaggacccatacactttcggaggcggcactaaggttgagatcaaa

SEQ ID NO: 306 - DNA, 333 bp, Artificial Sequence
  source: /note="Description of Artificial Sequence: Synthetic polynucleotide"
gagatagttatgactcagtctcccgccacactttcagtaagtcccggtgaacgcgccaccctgtcctgccgtgcttccgaatcagtggataatgacggcattaggtttttgcactggtaccaacaaaagcccggacaggccccccgcctgctgatatatcgtgcatcaacacgagcaacagggatccccgctcgatttagtggatccggaagcaggaccgaatttacacttaccatttcctcacttcagtcagaagatttcgccgtttactactgtcagcagtcaaataaggatccttacacatttgggggcggtacaaaagtcgagatcaaa

SEQ ID NO: 307 - DNA, 360 bp, Artificial Sequence
  source: /note="Description of Artificial Sequence: Synthetic polynucleotide"
gaggtccagttggtccagtcaggagccgaagtcaagaagcctggggaaagcctgaaaataagttgcaaagctagtggatatacatttacagattataccattcattgggtccggcaaatgccaggaaaaggcttggagtggatggggtggatttatcccctccgaggctcaataaattatagtcctagttttcaggggcaggtaactattagcgctgataaaagtatttctacagtttatttgcagtggagttcattgaaggctagtgacaccgctatgtatttctgcgctagacatggtgcatattattcaaatgccttcgactattggggccagggcaccctcgtcactgtgagttcc

SEQ ID NO: 308 - DNA, 360 bp, Artificial Sequence
  source: /note="Description of Artificial Sequence: Synthetic polynucleotide"
caggtgcaacttgttcagtcaggggctgaagtaaagaagccaggctcatcagtcaaggtatcatgcaaagcatctggctatacatttacagattacaccattcactgggtgaggcaagctcccggtcaaggtctcgagtggatggggtggatataccctctcagaggctctataaattacgctcagaaatttcaagggagagttacaattactgctgataaaagtaccagcactgcttatatggagctttcctcacttcgttcagaggacaccgccgtttacttttgtgcccggcatggtgcctattattcaaatgccttcgattattgggggcagggaactttggtcacagtttcatct

SEQ ID NO: 309 - DNA, 360 bp, Artificial Sequence
  source: /note="Description of Artificial Sequence: Synthetic polynucleotide"
caagttcaacttgtccaaagtggggctgaagttaaaaaacctggatcatcagtcaaggtttcatgcaaagccagcggttacacatttacagactatacaatacattgggttcgacaggctcccgggcaagggctcgaatggatgggatggatttatcccctcaggggctcaattaactatgctgagaaatttaagggtcgtgtaacactcaccgccgataaatccacctcaaccgtatatatggagctttcttctcttcgctctgaagataccgccgtctatttctgcgcacgacacggggcatactattctaatgcttttgactactggggacaagggacacttgtgaccgttagtagc

SEQ ID NO: 310 - DNA, 360 bp, Artificial Sequence
  source: /note="Description of Artificial Sequence: Synthetic polynucleotide"
caagtgcagttggtccagagtggagcagaggtgaagaagcctggtgcttccgtcaaggtgagttgcaaggcatctggttatactttcactgactacacaattcattgggtcaggcaggcccctggacagggactggaatggatgggatggatctatccacttagaggatcaatcaactatgctcaaaagttccagggtcgtgtaacaatgaccgcagacaaaagtatctcaactgtatacatggaattgtcccgattgaggagcgacgacacagccgtatattattgtgccaggcacggagcctactacagtaatgccttcgactactgggggcagggcacccttgttaccgtgtccagc

SEQ ID NO: 311 - DNA, 360 bp, Artificial Sequence
  source: /note="Description of Artificial Sequence: Synthetic polynucleotide"
caagtgcagctcgttcagtctggcgcagaagtgaagaagccaggagcttccgttaaagtgtcctgtaaagcctctggatatacattcacagattatacaattcactgggtgagacaagcaaccggtcaaggtctcgaatggatgggctggatataccccctccgaggttccatcaactacgctcaaaaattccaaggacgagtcactatgacagcaaacaagagttcctccactgtatatatggaactctctagtttgcgctctgaagacaccgccgtgtacttctgtgccaggcacggcgcatactattctaatgcatttgactattgggggcagggcacattggtaacagttagttcc

SEQ ID NO: 312 - DNA, 333 bp, Artificial Sequence
  source: /note="Description of Artificial Sequence: Synthetic polynucleotide"
gaaattgtaatgacccagagccccgccacccttagtgtgtccccaggcgagagggccactctttcttgccgcgcaagcgaatccgtagacaacgatggtataagatttttgcattggtatcagcaaaagccaggccaggcaccccggcttctcatctacagagctagcaccctcgaaactggaatccccgctcgtttttcaggatctggtagcggaacagaatttactttgacaattagtagtttgcagtcagaggactttgctgtctattattgccagcagtctaataaagatccatacaccttcggcggagggaccaaagtagagattaaa

SEQ ID NO: 313 - DNA, 360 bp, Artificial Sequence
  source: /note="Description of Artificial Sequence: Synthetic polynucleotide"
caagttcagttggtgcaaagcggggcagaagtgaagaaacctggtgcttctgtgaaagtttcctgcaaggccagcggctacacctttactgattacacaatacactgggtacggcaggcaactgggcaaggattggaatggatggggtggatatacccattgcgagggtctataaactacgcacagaaatttcaaggtcgagtaacaatgacagccgacaaatcaataagcaccgtttatatggaactctcatctctcaggagtgaggataccgccgtgtatttctgcgcacgacacggtgcatattactcaaacgctttcgactattggggccagggcacccttgtgactgttagtagc

SEQ ID NO: 314 - protein, 15 aa, Artificial Sequence
  source: /note="Description of Artificial Sequence: Synthetic peptide"
KSSQSVDNDGIRFLH

SEQ ID NO: 315 - protein, 7 aa, Artificial Sequence
  source: /note="Description of Artificial Sequence: Synthetic peptide"
RASTRES

SEQ ID NO: 316 - protein, 111 aa, Artificial Sequence
  source: /note="Description of Artificial Sequence: Synthetic polypeptide"
DIVMTQSPDSLAVSLGERATINCKSSQSVDNDGIRFLHWYQQKPGQPPKLLIYRASTRESGVPDRFSGSGSGTDFTLTISSLQAEDVAVYYCQQSNKDPYTFGGGTKVEIK

SEQ ID NO: 317 - protein, 120 aa, Artificial Sequence
  source: /note="Description of Artificial Sequence: Synthetic polypeptide"
QVQLVQSGAEVKKPGASVKVSCKASGYTFTDYTIHWVRQAPGQGLEWMGWIYPLRGSINYAQKFQGRVTLTADKSTSTVYMELSSLRSEDTAVYFCARHGAYYSNAFDYWGQGTLVTVSS

SEQ ID NO: 318 - DNA, 333 bp, Artificial Sequence
  source: /note="Description of Artificial Sequence: Synthetic polynucleotide"
gacattgtaatgacccagtctcccgatagcctcgctgtctcactcggagaacgcgcaaccatcaactgcaagtcctcccaaagcgttgacaatgacggcattaggtttttgcactggtaccagcagaaacccggtcaacctcctaagttgctcatttaccgagcatctacccgcgagtcaggagtacctgatcgcttttccggtagcggtagtggaacagattttactctgaccattagttcactccaggcagaagatgtggctgtctactactgccaacagtcaaataaagacccttataccttcggtgggggtaccaaagtagagatcaaa

SEQ ID NO: 319 - DNA, 360 bp, Artificial Sequence
  source: /note="Description of Artificial Sequence: Synthetic polynucleotide"
caggtgcagttggtccagagcggggcagaggttaagaagcctggggcctcagtaaaggtatcctgcaaggcttctgggtacaccttcacagattacactattcattgggtgcgccaagcacctggtcaaggccttgaatggatgggatggatttaccccttgcgagggagtattaattatgcacagaagttccagggaagggttactcttaccgccgacaagtccacatcaaccgtttacatggagctttcctctctcaggtccgaagacactgctgtatatttctgcgctcggcatggggcttattacagcaacgccttcgattactggggtcagggtacattggtcacagtgtccagt

SEQ ID NO: 320 - protein, 327 aa, Artificial Sequence
  source: /note="Description of Artificial Sequence: Synthetic polypeptide"
STKGPSVFPLAPSSKSTSGGTAALGCLVKDYFPEPVTVSWNSGALTSGVHTFPAVLQSSGLYSLSSVVTVPSSSLGTQTYICNVNHKPSNTKVDKKVEPKSCDKTHTCPPCPAPELLGGPSVFLFPPKPKDTLMISRTPEVTCVVVDVSHEDPEVKFNWYVDGVEVHNAKTKPREEQYNSTYRVVSVLTVLHQDWLNGKEYKCKVSNKALPAPIEKTISKAKGQPREPQVYTLPPSRDELTKNQVSLTCLVKGFYPSDIAVEWESNGQPENNYKTTPPVLDSDGSFFLYSKLTVDKSRWQQGNVFSCSVMHEALHNHYTQKSLSLSP

SEQ ID NO: 321 - protein, 328 aa, Artificial Sequence
  source: /note="Description of Artificial Sequence: Synthetic polypeptide"
ASTKGPSVFPLAPSSKSTSGGTAALGCLVKDYFPEPVTVSWNSGALTSGVHTFPAVLQSSGLYSLSSVVTVPSSSLGTQTYICNVNHKPSNTKVDKRVEPKSCDKTHTCPPCPAPELLGGPSVFLFPPKPKDTLMISRTPEVTCVVVDVSHEDPEVKFNWYVDGVEVHNAKTKPREEQYNSTYRVVSVLTVLHQDWLNGKEYKCKVSNKALPAPIEKTISKAKGQPREPQVYTLPPSREEMTKNQVSLTCLVKGFYPSDIAVEWESNGQPENNYKTTPPVLDSDGSFFLYSKLTVDKSRWQQGNVFSCSVMHEALHNHYTQKSLSLSP

SEQ ID NO: 322 - protein, 328 aa, Artificial Sequence
  source: /note="Description of Artificial Sequence: Synthetic polypeptide"
ASTKGPSVFPLAPSSKSTSGGTAALGCLVKDYFPEPVTVSWNSGALTSGVHTFPAVLQSSGLYSLSSVVTVPSSSLGTQTYICNVNHKPSNTKVDKKVEPKSCDKTHTCPPCPAPELLGGPSVFLFPPKPKDTLMISRTPEVTCVVVDVSHEDPEVKFNWYVDGVEVHNAKTKPREEQYNSTYRVVSVLTVLHQDWLNGKEYKCKVSNKALPAPIEKTISKAKGQPREPQVYTLPPSRDELTKNQVSLTCLVKGFYPSDIAVEWESNGQPENNYKTTPPVLDSDGSFFLYSKLTVDKSRWQQGNIFSCSVMHEALHNHYTQKSLSLSP

SEQ ID NO: 323 - protein, 323 aa, Artificial Sequence
  source: /note="Description of Artificial Sequence: Synthetic polypeptide"
STKGPSVFPLAPCSRSTSESTAALGCLVKDYFPEPVTVSWNSGALTSGVHTFPAVLQSSGLYSLSSVVTVPSSNFGTQTYTCNVDHKPSNTKVDKTVERKCCVECPPCPAPPVAGPSVFLFPPKPKDTLMISRTPEVTCVVVDVSHEDPEVQFNWYVDGVEVHNAKTKPREEQFNSTFRVVSVLTVVHQDWLNGKEYKCKVSNKGLPAPIEKTISKTKGQPREPQVYTLPPSREEMTKNQVSLTCLVKGFYPSDIAVEWESNGQPENNYKTTPPMLDSDGSFFLYSKLTVDKSRWQQGNVFSCSVMHEALHNHYTQKSLSLSP

SEQ ID NO: 324 - protein, 323 aa, Artificial Sequence
  source: /note="Description of Artificial Sequence: Synthetic polypeptide"
STKGPSVFPLAPCSRSTSESTAALGCLVKDYFPEPVTVSWNSGALTSGVHTFPAVLQSSGLYSLSSVVTVTSSNFGTQTYTCNVDHKPSNTKVDKTVERKCCVECPPCPAPPVAGPSVFLFPPKPKDTLMISRTPEVTCVVVDVSHEDPEVQFNWYVDGMEVHNAKTKPREEQFNSTFRVVSVLTVVHQDWLNGKEYKCKVSNKGLPAPIEKTISKTKGQPREPQVYTLPPSREEMTKNQVSLTCLVKGFYPSDIAVEWESNGQPENNYKTTPPMLDSDGSFFLYSKLTVDKSRWQQGNVFSCSVMHEALHNHYTQKSLSLSP

SEQ ID NO: 325 - protein, 323 aa, Artificial Sequence
  source: /note="Description of Artificial Sequence: Synthetic polypeptide"
STKGPSVFPLAPCSRSTSESTAALGCLVKDYFPEPVTVSWNSGALTSGVHTFPAVLQSSGLYSLSSVVTVPSSSLGTQTYTCNVDHKPSNTKVDKTVERKCCVECPPCPAPPVAGPSVFLFPPKPKDTLMISRTPEVTCVVVDVSHEDPEVQFNWYVDGVEVHNAKTKPREEQFNSTFRVVSVLTVVHQDWLNGKEYKCKVSNKGLPAPIEKTISKTKGQPREPQVYTLPPSREEMTKNQVSLTCLVKGFYPSDIAVEWESNGQPENNYKTTPPMLDSDGSFFLYSKLTVDKSRWQQGNVFSCSVMHEALHNHYTQKSLSLSP

SEQ ID NO: 326 - protein, 323 aa, Artificial Sequence
  source: /note="Description of Artificial Sequence: Synthetic polypeptide"
STKGPSVFPLAPCSRSTSESTAALGCLVKDYFPEPVTVSWNSGALTSGVHTFPAVLQSSGLYSLSSVVTVPSSNFGTQTYTCNVDHKPSNTKVDKTVERKCCVECPPCPAPPVAGPSVFLFPPKPKDTLMISRTPEVTCVVVDVSHEDPEVQFNWYVDGVEVHNAKTKPREEQFNSTFRVVSVLTVVHQDWLNGKEYKCKVSNKGLPAPIEKTISKTKGQPREPQVYTLPPSREEMTKNQVSLTCLVKGFYPSDISVEWESNGQPENNYKTTPPMLDSDGSFFLYSKLTVDKSRWQQGNVFSCSVMHEALHNHYTQKSLSLSP

SEQ ID NO: 327 - protein, 15 aa, Artificial Sequence
  source: /note="Description of Artificial Sequence: Synthetic peptide"
  VARIANT (1)..(1): /replace="Lys"
  VARIANT (2)..(2): /replace="Ser"
  VARIANT (4)..(4): /replace="Gln"
  VARIANT (14)..(14): /replace="Leu"
  MISC_FEATURE (1)..(15): /note="Variant residues given in the sequence have no preference with respect to those in the annotations for variant positions"
RASESVDNDGIRFMH

SEQ ID NO: 328 - protein, 7 aa, Artificial Sequence
  source: /note="Description of Artificial Sequence: Synthetic peptide"
  VARIANT (4)..(4): /replace="Thr"
  VARIANT (5)..(5): /replace="Arg"
  VARIANT (6)..(6): /replace="Ala"
  VARIANT (7)..(7): /replace="Thr"
  MISC_FEATURE (1)..(7): /note="Variant residues given in the sequence have no preference with respect to those in the annotations for variant positions"
RASNLES

SEQ ID NO: 329 - protein, 17 aa, Artificial Sequence
  source: /note="Description of Artificial Sequence: Synthetic peptide"
  VARIANT (12)..(12): /replace="Ser" or "Ala"
  VARIANT (13)..(13): /replace="Pro" or "Gln"
  VARIANT (14)..(14): /replace="Ser"
  VARIANT (16)..(16): /replace="Gln"
  VARIANT (17)..(17): /replace="Gly"
  MISC_FEATURE (1)..(17): /note="Variant residues given in the sequence have no preference with respect to those in the annotations for variant positions"
WIYPLRGSINYNEKFKD

SEQ ID NO: 330 - protein, 8 aa, Artificial Sequence
  source: /note="Description of Artificial Sequence: Synthetic peptide"
  VARIANT (3)..(3): /replace="Thr"
  VARIANT (4)..(4): /replace="Phe"
  VARIANT (6)..(6): /replace=" "
  VARIANT (7)..(7): /replace="Asp" or "Ser"
  MISC_FEATURE (1)..(8): /note="Variant residues given in the sequence have no preference with respect to those in the annotations for variant positions"
GYSITSGY

SEQ ID NO: 331 - protein, 6 aa, Artificial Sequence
  source: /note="Description of Artificial Sequence: Synthetic peptide"
  VARIANT (1)..(1): /replace="Tyr" or " "
  VARIANT (2)..(2): /replace="Pro"
  VARIANT (3)..(3): /replace="Leu" or "Arg"
  VARIANT (4)..(4): /replace="Asn" or "Arg"
  VARIANT (5)..(5): /replace="Ser"
  VARIANT (6)..(6): /replace="Asp" or "Ser"
  MISC_FEATURE (1)..(6): /note="Variant residues given in the sequence have no preference with respect to those in the annotations for variant positions"
NSYDGY

SEQ ID NO: 332 - protein, 12 aa, Artificial Sequence
  source: /note="Description of Artificial Sequence: Synthetic peptide"
  VARIANT (1)..(1): /replace="Glu" or "His"
  VARIANT (2)..(2): /replace=" "
  VARIANT (3)..(3): /replace="Asp" or "Ala"
  VARIANT (4)..(4): /replace="Gly" or "Tyr"
  VARIANT (6)..(6): /replace="Asp" or " "
  VARIANT (7)..(7): /replace="Tyr" or "Ser" or "Lys"
  VARIANT (8)..(8): /replace="Asn" or "Arg"
  VARIANT (9)..(9): /replace="Ala" or "Gly"
  VARIANT (11)..(11): /replace="Asp"
  VARIANT (12)..(12): /replace="Tyr"
  MISC_FEATURE (1)..(12): /note="Variant residues given in the sequence have no preference with respect to those in the annotations for variant positions"
YGYDYEDWYFGV

SEQ ID NO: 333 - protein, 15 aa, Artificial Sequence
  source: /note="Description of Artificial Sequence: Synthetic peptide"
  VARIANT (1)..(1): /replace="Lys"
  VARIANT (4)..(4): /replace="Gln"
  VARIANT (7)..(7): /replace="Ser"
  VARIANT (8)..(8): /replace="Phe" or "Ile"
  VARIANT (9)..(9): /replace="Ala" or "Ile" or "Asp"
  VARIANT (11)..(11): /replace="Thr"
  VARIANT (12)..(12): /replace="Asn" or "Arg"
  VARIANT (13)..(13): /replace="Leu" or "Ser"
  VARIANT (14)..(14): /replace="Ile"
  VARIANT (15)..(15): /replace="His"
  MISC_FEATURE (1)..(15): /note="Variant residues given in the sequence have no preference with respect to those in the annotations for variant positions"
RASESVDNYGISFMN

SEQ ID NO: 334 - protein, 7 aa, Artificial Sequence
  source: /note="Description of Artificial Sequence: Synthetic peptide"
  VARIANT (1)..(1): /replace="Arg" or "His"
  VARIANT (5)..(5): /replace="Leu"
  VARIANT (6)..(6): /replace="Glu"
  VARIANT (7)..(7): /replace="Pro" or "Thr"
  MISC_FEATURE (1)..(7): /note="Variant residues given in the sequence have no preference with respect to those in the annotations for variant positions"
AASNQGS

SEQ ID NO: 335 - protein, 9 aa, Artificial Sequence
  source: /note="Description of Artificial Sequence: Synthetic peptide"
  VARIANT (1)..(1): /replace="Leu"
  VARIANT (4)..(4): /replace="Arg" or "Asn"
  VARIANT (5)..(5): /replace="Lys"
  VARIANT (6)..(6): /replace="Tyr" or "Ile" or "Asp"
  VARIANT (8)..(8): /replace="Trp" or "Tyr"
  MISC_FEATURE (1)..(9): /note="Variant residues given in the sequence have no preference with respect to those in the annotations for variant positions"
QQSKEVPRT

SEQ ID NO: 336 - protein, 6 aa, Artificial Sequence
  source: /note="Description of Artificial Sequence: Synthetic peptide"
  VARIANT (1)..(1): /replace=" "
  VARIANT (2)..(2): /replace="Asp" or "Ser"
  VARIANT (4)..(4): /replace="Phe" or "Thr" or "Asp"
  VARIANT (5)..(5): /replace="Met" or "Ile" or "Val"
  VARIANT (6)..(6): /replace="His" or "Phe"
  MISC_FEATURE (1)..(6): /note="Variant residues given in the sequence have no preference with respect to those in the annotations for variant positions"
SGYYWN

SEQ ID NO: 337 - protein, 17 aa, Artificial Sequence
  source: /note="Description of Artificial Sequence: Synthetic peptide"
  VARIANT (1)..(1): /replace="Arg or "Trp"
  VARIANT (3)..(3): /replace="Tyr" or " "
  VARIANT (4)..(4): /replace="Pro"
  VARIANT (5)..(5): /replace="Leu" or "Arg"
  VARIANT (6)..(6): /replace="Asn" or "Arg"
  VARIANT (7)..(7): /replace="Ser"
  VARIANT (8)..(8): /replace="Asp" or "Ser"
  VARIANT (9)..(9): /replace="Thr" or "Ile"
  VARIANT (10)..(10): /replace="Phe" or "Lys"
  VARIANT (13)..(13): /replace="Gln" or "Glu"
  VARIANT (14)..(14): /replace="Lys"
  VARIANT (15)..(15): /replace="Phe"
  VARIANT (17)..(17): /replace="Gly" or "Asp"
  MISC_FEATURE (1)..(17): /note="Variant residues given in the sequence have no preference with respect to those in the annotations for variant positions"
YINSYDGYNNYNPSLKN

SEQ ID NO: 338 - protein, 4 aa, Artificial Sequence
  source: /note="Description of Artificial Sequence: Synthetic peptide"
DDSD

SEQ ID NO: 339 - protein, 8 aa, Artificial Sequence
  source: /note="Description of Artificial Sequence: Synthetic peptide"
VTFTMGQV

SEQ ID NO: 340 - protein, 4 aa, Artificial Sequence
  source: /note="Description of Artificial Sequence: Synthetic peptide"
MPSH

SEQ ID NO: 341 - protein, 4 aa, Artificial Sequence
  source: /note="Description of Artificial Sequence: Synthetic peptide"
PRAR

SEQ ID NO: 342 - protein, 16 aa, Artificial Sequence
  source: /note="Description of Artificial Sequence: Synthetic peptide"
  VARIANT (12)..(12): /replace="Pro"
  VARIANT (13)..(13): /replace="Ser"
  VARIANT (14)..(14): /replace="Leu"
  VARIANT (15)..(15): /replace="Lys"
  MISC_FEATURE (1)..(16): /note="Variant residues given in the sequence have no preference with respect to those in the annotations for variant positions"
VIWSDGSTDYNAAFIS

SEQ ID NO: 343 - protein, 5 aa, Artificial Sequence
  source: /note="Description of Artificial Sequence: Synthetic peptide"
  VARIANT (4)..(4): /replace="Met"
  MISC_FEATURE (1)..(5): /note="Variant residues given in the sequence have no preference with respect to those in the annotations for variant positions"
DYYIN

SEQ ID NO: 344 - protein, 17 aa, Artificial Sequence
  source: /note="Description of Artificial Sequence: Synthetic peptide"
  VARIANT (12)..(12): /replace="Ala"
  VARIANT (13)..(13): /replace="Gln"
  VARIANT (15)..(15): /replace="Leu"
  VARIANT (16)..(16): /replace="Gln"
  MISC_FEATURE (1)..(17): /note="Variant residues given in the sequence have no preference with respect to those in the annotations for variant positions"
WIFPGSGSTYYNEKFKG

SEQ ID NO: 345 - protein, 11 aa, Artificial Sequence
  source: /note="Description of Artificial Sequence: Synthetic peptide"
  VARIANT (1)..(1): /replace="Gln"
  MISC_FEATURE (1)..(11): /note="Variant residues given in the sequence have no preference with respect to those in the annotations for variant positions"
KASQDINKYIA

SEQ ID NO: 346 - protein, 7 aa, Artificial Sequence
  source: /note="Description of Artificial Sequence: Synthetic peptide"
  VARIANT (6)..(6): /replace="Glu"
  VARIANT (7)..(7): /replace="Thr"
  MISC_FEATURE (1)..(7): /note="Variant residues given in the sequence have no preference with respect to those in the annotations for variant positions"
YTSTLQS